European Patent Application EP 4 534 097 A1, published April 9, 2025. Title: Composition for Treating Retinal or Macular Disease. Applicant: NEURACLE GENETICS INC. The sequence listing filed with the application follows.

SEQUENCE LISTING (313 sequences)

SEQ ID NO: 1 - DNA, 924 bp, synthetic construct
  misc_feature 1..924: note = EF-1 alpha intron FL
  source 1..924: mol_type = other DNA
cccgcgggcctggcctctttacgggttatggcccttgcgtgccttgaattacttccacgcccctggctgcagtacgtgattcttgatcccgagcttcgggttggaagtgggtgggagagttcgaggccttgcgcttaaggagccccttcgcctcgtgcttgagttgaggcctggcttgggcgctggggccgccgcgtgcgaatctggtggcaccttcgcgcctgtctcgctgctttcgataagtctctagccatttaaaatttttgatgacctgctgcgacgctttttttctggcaagatagtcttgtaaatgcgggccaagatctgcacactggtatttcggtttttggggccgcgggcggcgacggggcccgtgcgtcccagcgcacatgttcggcgaggcggggcctgcgagcgcggccaccgagaatcggacgggggtagtctcaagctggccggcctgctctggtgcctggcctcgcgccgccgtgtatcgccccgccctgggcggcaaggctggcccggtcggcaccagttgcgtgagcggaaagatggccgcttcccggccctgctgcagggagctcaaaatggaggacgcggcgctcgggagagcgggcgggtgagtcacccacacaaaggaaaagggcctttccgtcctcagccgtcgcttcatgtgactccacggagtaccgggcgccgtccaggcacctcgattagttctcgagcttttggagtacgtcgtctttaggttggggggaggggttttatgcgatggagtttccccacactgagtgggtggagactgaagttaggccagcttggcacttgatgtaattctccttggaatttgccctttttgagtttggatcttggttcattctcaagcctcagacagtggttcaaagtttttttcttccatttcag

SEQ ID NO: 2 - DNA, 95 bp, synthetic construct
  misc_feature 1..95: note = EF-1 alpha intron fragment T3.1.1
  source 1..95: mol_type = other DNA
tgtaattctccttggaatttgccctttttgagtttggatcttggttcattctcaagcctcagacagtggttcaaagtttttttcttccatttcag

SEQ ID NO: 3 - DNA, 73 bp, synthetic construct
  misc_feature 1..73: note = EF-1 alpha intron fragment T3.1.2
  source 1..73: mol_type = other DNA
cctttttgagtttggatcttggttcattctcaagcctcagacagtggttcaaagtttttttcttccatttcag

SEQ ID NO: 4 - DNA, 380 bp, synthetic construct
  misc_feature 1..380: note = CMV enhancer
  source 1..380: mol_type = other DNA
gacattgattattgactagttattaatagtaatcaattacggggtcattagttcatagcccatatatggagttccgcgttacataacttacggtaaatggcccgcctggctgaccgcccaacgacccccgcccattgacgtcaataatgacgtatgttcccatagtaacgccaatagggactttccattgacgtcaatgggtggagtatttacggtaaactgcccacttggcagtacatcaagtgtatcatatgccaagtacgccccctattgacgtcaatgacggtaaatggcccgcctggcattatgcccagtacatgaccttatgggactttcctacttggcagtacatctacgtattagtcatcgctattaccatg

SEQ ID NO: 5 - DNA, 31 bp, synthetic construct
  misc_feature 1..31: note = CMV promoter fragment
  source 1..31: mol_type = other DNA
gtgatgcggttttggcagtacaccaatgggc

SEQ ID NO: 6 - DNA, 218 bp, synthetic construct
  misc_feature 1..218: note = CMV promoter
  source 1..218: mol_type = other DNA
gtgatgcggttttggcagtacatcaatgggcgtggatagcggtttgactcacggggatttccaagtctccaccccattgacgtcaatgggagtttgttttggcaccaaaatcaacgggactttccaaaatgtcgtaacaactccgccccattgacgcaaatgggcggtaggcgtgtacggtgggaggtctatataagcagagctcgtttagtgaaccg

SEQ ID NO: 7 - DNA, 201 bp, synthetic construct
  misc_feature 1..201: note = EF-1 alpha promoter
  source 1..201: mol_type = other DNA
gctccggtgcccgtcagtgggcagagcgcacatcgcccacagtccccgagaagttggggggaggggtcggcaattgaaccggtgcctagagaaggtggcgcggggtaaactgggaaagtgatgtcgtgtactggctccgcctttttcccgagggtgggggagaaccgtatataagtgcagtagtcgccgtgaacgttcttt

SEQ ID NO: 8 - DNA, 279 bp, synthetic construct
  misc_feature 1..279: note = Chicken beta-actin promoter
  source 1..279: mol_type = other DNA
gtcgaggtgagccccacgttctgcttcactctccccatctcccccccctccccacccccaattttgtatttatttattttttaattattttgtgcagcgatgggggcggggggggggggggggcgcgcgccaggcggggcggggcggggcgaggggcggggcggggcgaggcggagaggtgcggcggcagccaatcagagcggcgcgctccgaaagtttccttttatggcgaggcggcggcggcggcggccctataaaaagcgaagcgcgcggcgggcg

SEQ ID NO: 9 - DNA, 19 bp, synthetic construct
  misc_feature 1..19: note = EF-1 alpha splicing donor
  source 1..19: mol_type = other DNA
gtaagtgccgtgtgtggtt

SEQ ID NO: 10 - DNA, 43 bp, synthetic construct
  misc_feature 1..43: note = Chicken beta-actin splicing donor
  source 1..43: mol_type = other DNA
gtgagcgggcgggacggcccttctcctccgggctgtaattagc

SEQ ID NO: 11 - skipped

SEQ ID NO: 12 - DNA, 30 bp, synthetic construct
  misc_feature 1..30: note = CMV exon 1 fragment
  source 1..30: mol_type = other DNA
tcagatcgcctggagacgccatccacgctg

SEQ ID NO: 13 - DNA, 29 bp, synthetic construct
  misc_feature 1..29: note = EF-1 alpha exon 1 fragment
  source 1..29: mol_type = other DNA
ttcgcaacgggtttgccgccagaacacag

SEQ ID NO: 14 - DNA, 32 bp, synthetic construct
  misc_feature 1..32: note = Chicken beta-actin exon 1 fragment 1
  source 1..32: mol_type = other DNA
ggagtcgctgcgcgctgccttcgccccgtgcc

SEQ ID NO: 15 - DNA, 93 bp, synthetic construct
  misc_feature 1..93: note = Chicken beta-actin exon 1 fragment 2
  source 1..93: mol_type = other DNA
ggagtcgctgcgcgctgccttcgccccgtgccccgctccgccgccgcctcgcgccgcccgccccggctctgactgaccgcgttactcccacag

SEQ ID NO: 16 - DNA, 23 bp, synthetic construct
  misc_feature 1..23: note = miR142-3p target sequence
  source 1..23: mol_type = other DNA
tccataaagtaggaaacactaca

SEQ ID NO: 17 - DNA, 104 bp, synthetic construct
  misc_feature 1..104: note = Four repeats of miR142-3p target sequence with spacer
  source 1..104: mol_type = other DNA
tccataaagtaggaaacactacacgattccataaagtaggaaacactacaacgttccataaagtaggaaacactacatcactccataaagtaggaaacactaca

SEQ ID NO: 18 - DNA, 589 bp, synthetic construct
  misc_feature 1..589: note = WPRE
  source 1..589: mol_type = other DNA
aatcaacctctggattacaaaatttgtgaaagattgactggtattcttaactatgttgctccttttacgctatgtggatacgctgctttaatgcctttgtatcatgctattgcttcccgtatggctttcattttctcctccttgtataaatcctggttgctgtctctttatgaggagttgtggcccgttgtcaggcaacgtggcgtggtgtgcactgtgtttgctgacgcaacccccactggttggggcattgccaccacctgtcagctcctttccgggactttcgctttccccctccctattgccacggcggaactcatcgccgcctgccttgcccgctgctggacaggggctcggctgttgggcactgacaattccgtggtgttgtcggggaagctgacgtcctttccatggctgctcgcctgtgttgccacctggattctgcgcgggacgtccttctgctacgtcccttcggccctcaatccagcggaccttccttcccgcggcctgctgccggctctgcggcctcttccgcgtcttcgccttcgccctcagacgagtcggatctccctttgggccgcctccccgc

SEQ ID NO: 19 - DNA, 477 bp, synthetic construct
  misc_feature 1..477: note = hGH pA sequence
  source 1..477: mol_type = other DNA
gggtggcatccctgtgacccctccccagtgcctctcctggccctggaagttgccactccagtgcccaccagccttgtcctaataaaattaagttgcatcattttgtctgactaggtgtccttctataatattatggggtggaggggggtggtatggagcaaggggcaagttgggaagacaacctgtagggcctgcggggtctattgggaaccaagctggagtgcagtggcacaatcttggctcactgcaatctccgcctcctgggttcaagcgattctcctgcctcagcctcccgagttgttgggattccaggcatgcatgaccaggctcagctaatttttgtttttttggtagagacggggtttcaccatattggccaggctggtctccaactcctaatctcaggtgatctacccaccttggcctcccaaattgctgggattacaggcgtgaaccactgctcccttccctgtcctt

SEQ ID NO: 20 - DNA, 225 bp, synthetic construct
  misc_feature 1..225: note = bGH pA sequence
  source 1..225: mol_type = other DNA
ctgtgccttctagttgccagccatctgttgtttgcccctcccccgtgccttccttgaccctggaaggtgccactcccactgtcctttcctaataaaatgaggaaattgcatcgcattgtctgagtaggtgtcattctattctggggggtggggtggggcaggacagcaagggggaggattgggaagacaatagcaggcatgctggggatgcggtgggctctatgg

SEQ ID NO: 21 - DNA, 122 bp, synthetic construct
  misc_feature 1..122: note = SV40 early pA sequence
  source 1..122: mol_type = other DNA
aacttgtttattgcagcttataatggttacaaataaagcaatagcatcacaaatttcacaaataaagcatttttttcactgcattctagttgtggtttgtccaaactcatcaatgtatctta

SEQ ID NO: 22 - DNA, 134 bp, synthetic construct
  misc_feature 1..134: note = SV40 late pA sequence
  source 1..134: mol_type = other DNA
atgctttatttgtgaaatttgtgatgctattgctttatttgtaaccattataagctgcaataaacaagttaacaacaacaattgcattcattttatgtttcaggttcagggggaggtgtgggaggttttttaaa

SEQ ID NO: 23 - DNA, 1296 bp, synthetic construct
  misc_feature 1..1296: note = Aflibercept
  source 1..1296: mol_type = other DNA
tctgataccggcagacccttcgtggaaatgtacagcgagatccccgagatcatccacatgaccgagggcagagagctggtcatcccttgcagagtgacaagccccaacatcaccgtgacactgaagaagttccctctggacacactgatccccgacggcaagagaatcatctgggacagccggaagggcttcatcatcagcaacgccacctacaaagagatcggcctgctgacatgcgaggccacagtgaatggccacctgtacaagaccaactacctgacacacagacagaccaacaccatcatcgacgtggtgctgagcccttctcacggcattgagctgtctgtgggagagaagctggtgctgaattgcaccgccagaaccgagctgaacgtgggcatcgacttcaactgggagtaccccagcagcaagcaccagcacaagaaactggtcaaccgggacctgaaaacccagagcggcagcgagatgaagaaattcctgagcaccctgaccatcgacggcgtgacaagaagcgatcagggcctgtacacatgtgccgccagctctggcctgatgaccaagaaaaacagcaccttcgtgcgggtgcacgagaaggacaagacccacacatgtcctccatgtcctgctccagaactgctcggcggaccctccgttttcctgtttccacctaagcctaaggacaccctgatgatcagcagaacccctgaagtgacctgcgtggtggtggatgtgtctcacgaggaccccgaagtgaagttcaattggtacgtggacggcgtggaagtgcacaacgccaagaccaagcctagagaggaacagtacaactccacatacagagtggtgtccgtgctgaccgtgctgcaccaggattggctgaacggcaaagagtacaagtgcaaggtgtccaacaaggccctgcctgctcctatcgagaaaaccatctccaaggccaagggccagccaagagaaccccaggtttacacactgcctccaagcagggacgagctgacaaagaatcaggtgtccctgacctgcctggtcaagggcttctacccttccgatatcgccgtggaatgggagagcaatggccagcctgagaacaactacaagacaacccctcctgtgctggacagcgacggctcattcttcctgtacagcaagctgacagtggacaagagcagatggcagcagggcaacgtgttcagctgttctgtgatgcacgaggccctgcacaaccactacacccagaagtctctgagcttgtctcctggctaa

SEQ ID NO: 24 - DNA, 30 bp, synthetic construct
  misc_feature 1..30: note = Oligo #001
  source 1..30: mol_type = other DNA
ggaagatctctgtgccttctagttgccagc

SEQ ID NO: 25 - DNA, 31 bp, synthetic construct
  misc_feature 1..31: note = Oligo #002
  source 1..31: mol_type = other DNA
cacgtggttaccccatagagcccaccgcatc

SEQ ID NO: 26 - DNA, 61 bp, synthetic construct
  misc_feature 1..61: note = Oligo #003
  source 1..61: mol_type = other DNA
agctttccataaagtaggaaacactacacgattccataaagtaggaaacactacaacgttc

SEQ ID NO: 27 - DNA, 48 bp, synthetic construct
  misc_feature 1..48: note = Oligo #004
  source 1..48: mol_type = other DNA
tagtgtttcctactttatggaatcgtgtagtgtttcctactttatgga

SEQ ID NO: 28 - DNA, 49 bp, synthetic construct
  misc_feature 1..49: note = Oligo #005
  source 1..49: mol_type = other DNA
cataaagtaggaaacactacatcactccataaagtaggaaacactacag

SEQ ID NO: 29 - DNA, 61 bp, synthetic construct
  misc_feature 1..61: note = Oligo #006
  source 1..61: mol_type = other DNA
tcgactgtagtgtttcctactttatggagtgatgtagtgtttcctactttatggaacgttg

SEQ ID NO: 30 - DNA, 31 bp, synthetic construct
  misc_feature 1..31: note = Oligo #007
  source 1..31: mol_type = other DNA
gtgtgtggtttgctgcagggagctcaaaatg

SEQ ID NO: 31 - DNA, 20 bp, synthetic construct
  misc_feature 1..20: note = Oligo #008
  source 1..20: mol_type = other DNA
cggtgatgacggtgaaaacc

SEQ ID NO: 32 - DNA, 30 bp, synthetic construct
  misc_feature 1..30: note = Oligo #009
  source 1..30: mol_type = other DNA
ccctgcagcaaaccacacacggcacttacc

SEQ ID NO: 33 - DNA, 20 bp, synthetic construct
  misc_feature 1..20: note = Oligo #010
  source 1..20: mol_type = other DNA
ggttttcaccgtcatcaccg

SEQ ID NO: 34 - DNA, 31 bp, synthetic construct
  misc_feature 1..31: note = Oligo #011
  source 1..31: mol_type = other DNA
gtgtgtggtttcgagcttttggagtacgtcg

SEQ ID NO: 35 - DNA, 30 bp, synthetic construct
  misc_feature 1..30: note = Oligo #012
  source 1..30: mol_type = other DNA
aaaagctcgaaaccacacacggcacttacc

SEQ ID NO: 36 - DNA, 28 bp, synthetic construct
  misc_feature 1..28: note = Oligo #013
  source 1..28: mol_type = other DNA
gtgtgtggttgttaggccagcttggcac

SEQ ID NO: 37 - DNA, 30 bp, synthetic construct
  misc_feature 1..30: note = Oligo #014
  source 1..30: mol_type = other DNA
ctggcctaacaaccacacacggcacttacc

SEQ ID NO: 38 - DNA, 33 bp, synthetic construct
  misc_feature 1..33: note = Oligo #015
  source 1..33: mol_type = other DNA
gtgtgtggtttcattctcaagcctcagacagtg

SEQ ID NO: 39 - DNA, 30 bp, synthetic construct
  misc_feature 1..30: note = Oligo #016
  source 1..30: mol_type = other DNA
ttgagaatgaaaccacacacggcacttacc

SEQ ID NO: 40 - DNA, 40 bp, synthetic construct
  misc_feature 1..40: note = Oligo #017
  source 1..40: mol_type = other DNA
gtgtgtggtttggttcaaagtttttttcttccatttcagg

SEQ ID NO: 41 - DNA, 30 bp, synthetic construct
  misc_feature 1..30: note = Oligo #018
  source 1..30: mol_type = other DNA
ctttgaaccaaaccacacacggcacttacc

SEQ ID NO: 42 - DNA, 52 bp, synthetic construct
  misc_feature 1..52: note = Oligo #019
  source 1..52: mol_type = other DNA
ccggaattctgacattgattattgactagttattaatagtaatcaattacgg

SEQ ID NO: 43 - DNA, 28 bp, synthetic construct
  misc_feature 1..28: note = Oligo #020
  source 1..28: mol_type = other DNA
cgcggatccctgtgttctggcggcaaac

SEQ ID NO: 44 - DNA, 39 bp, synthetic construct
  misc_feature 1..39: note = Oligo #021
  source 1..39: mol_type = other DNA
cgcggatcccggttcactaaacgagctctgcttatatag

SEQ ID NO: 45 - DNA, 30 bp, synthetic construct
  misc_feature 1..30: note = Oligo #022
  source 1..30: mol_type = other DNA
tgtaattctccttggaatttgccctttttg

SEQ ID NO: 46 - DNA, 32 bp, synthetic construct
  misc_feature 1..32: note = Oligo #023
  source 1..32: mol_type = other DNA
cccaagcttggatcctcacgacacctgaaatg

SEQ ID NO: 47 - DNA, 89 bp, synthetic construct
  misc_feature 1..89: note = Oligo #024
  source 1..89: mol_type = other DNA
cctttttgagtttggatcttggttcattctcaagcctcagacagtggttcaaagtttttttcttccatttcaggtgtcgtgaggatcca

SEQ ID NO: 48 - DNA, 93 bp, synthetic construct
  misc_feature 1..93: note = Oligo #025
  source 1..93: mol_type = other DNA
agcttggatcctcacgacacctgaaatggaagaaaaaaactttgaaccactgtctgaggcttgagaatgaaccaagatccaaactcaaaaagg

SEQ ID NO: 49 - DNA, 27 bp, synthetic construct
  misc_feature 1..27: note = Oligo #026
  source 1..27: mol_type = other DNA
cggggtaccttcgcaacgggtttgccg

SEQ ID NO: 50 - DNA, 21 bp, synthetic construct
  misc_feature 1..21: note = Oligo #027
  source 1..21: mol_type = other DNA
cgcggatcctcacgacacctg

SEQ ID NO: 51 - DNA, 26 bp, synthetic construct
  misc_feature 1..26: note = Oligo #028
  source 1..26: mol_type = other DNA
tgaggatccgccaccatggagtttgg

SEQ ID NO: 52 - DNA, 49 bp, synthetic construct
  misc_feature 1..49: note = Oligo #029
  source 1..49: mol_type = other DNA
cgcaagcttcagtagcgctttagccaggagacaagctcagagacttctg

SEQ ID NO: 53 - DNA, 21 bp, synthetic construct
  misc_feature 1..21: note = Oligo #030
  source 1..21: mol_type = other DNA
ggaacccctagtgatggagtt

SEQ ID NO: 54 - DNA, 16 bp, synthetic construct
  misc_feature 1..16: note = Oligo #031
  source 1..16: mol_type = other DNA
cggcctcagtgagcga

SEQ ID NO: 55 - DNA, 21 bp, synthetic construct
  misc_feature 1..21: note = Oligo #032
  source 1..21: mol_type = other DNA
cactccctctctgcgcgctcg

SEQ ID NO: 56 - DNA, 57 bp, synthetic construct
  misc_feature 1..57: note = hIgG signal peptide sequence
  source 1..57: mol_type = other DNA
atggagtttgggctgagctgggttttcctcgttgctctttttagaggtgtccagtgt

SEQ ID NO: 57 - DNA, 51 bp, synthetic construct
  misc_feature 1..51: note = EF-1 alpha intron fragment T3.2
  source 1..51: mol_type = other DNA
ttcattctcaagcctcagacagtggttcaaagtttttttcttccatttcag

SEQ ID NO: 58 - DNA, 54 bp, synthetic construct
  misc_feature 1..54: note = EF-1 alpha intron fragment
  source 1..54: mol_type = other DNA
tggttcattctcaagcctcagacagtggttcaaagtttttttcttccatttcag

SEQ ID NO: 59 - DNA, 64 bp, synthetic construct
  misc_feature 1..64: note = EF-1 alpha intron fragment
  source 1..64: mol_type = other DNA
gtttggatcttggttcattctcaagcctcagacagtggttcaaagtttttttcttccatttcag

SEQ ID NO: 60 - DNA, 73 bp, synthetic construct; identical to SEQ ID NO: 3
  misc_feature 1..73: note = EF-1 alpha intron fragment
  source 1..73: mol_type = other DNA

SEQ ID NO: 61 - DNA, 74 bp, synthetic construct
  misc_feature 1..74: note = EF-1 alpha intron fragment
  source 1..74: mol_type = other DNA
ccctttttgagtttggatcttggttcattctcaagcctcagacagtggttcaaagtttttttcttccatttcag

SEQ ID NO: 62 - DNA, 84 bp, synthetic construct
  misc_feature 1..84: note = EF-1 alpha intron fragment
  source 1..84: mol_type = other DNA
ttggaatttgccctttttgagtttggatcttggttcattctcaagcctcagacagtggttcaaagtttttttcttccatttcag

SEQ ID NO: 63 - DNA, 104 bp, synthetic construct
  misc_feature 1..104: note = EF-1 alpha intron fragment
  source 1..104: mol_type = other DNA
ggcacttgatgtaattctccttggaatttgccctttttgagtttggatcttggttcattctcaagcctcagacagtggttcaaagtttttttcttccatttcag

SEQ ID NO: 64 - DNA, 114 bp, synthetic construct
  misc_feature 1..114: note = EF-1 alpha intron fragment
  source 1..114: mol_type = other DNA
aggccagcttggcacttgatgtaattctccttggaatttgccctttttgagtttggatcttggttcattctcaagcctcagacagtggttcaaagtttttttcttccatttcag

SEQ ID NO: 65 - DNA, 117 bp, synthetic construct
  misc_feature 1..117: note = EF-1 alpha intron fragment
  source 1..117: mol_type = other DNA
gttaggccagcttggcacttgatgtaattctccttggaatttgccctttttgagtttggatcttggttcattctcaagcctcagacagtggttcaaagtttttttcttccatttcag

SEQ ID NO: 66 - DNA, 124 bp, synthetic construct
  misc_feature 1..124: note = EF-1 alpha intron fragment
  source 1..124: mol_type = other DNA
gactgaagttaggccagcttggcacttgatgtaattctccttggaatttgccctttttgagtttggatcttggttcattctcaagcctcagacagtggttcaaagtttttttcttccatttcag

SEQ ID NO: 67 - DNA, 174 bp, synthetic construct
  misc_feature 1..174: note = EF-1 alpha intron fragment
  source 1..174: mol_type = other DNA
tggggggaggggttttatgcgatggagtttccccacactgagtgggtggagactgaagttaggccagcttggcacttgatgtaattctccttggaatttgccctttttgagtttggatcttggttcattctcaagcctcagacagtggttcaaagtttttttcttccatttcag

SEQ ID NO: 68 - DNA, 204 bp, synthetic construct
  misc_feature 1..204: note = EF-1 alpha intron fragment
  source 1..204: mol_type = other DNA
tcgagcttttggagtacgtcgtctttaggttggggggaggggttttatgcgatggagtttccccacactgagtgggtggagactgaagttaggccagcttggcacttgatgtaattctccttggaatttgccctttttgagtttggatcttggttcattctcaagcctcagacagtggttcaaagtttttttcttccatttcag

SEQ ID NO: 69 - DNA, 224 bp, synthetic construct
  misc_feature 1..224: note = EF-1 alpha intron fragment
  source 1..224: mol_type = other DNA
ccaggcacctcgattagttctcgagcttttggagtacgtcgtctttaggttggggggaggggttttatgcgatggagtttccccacactgagtgggtggagactgaagttaggccagcttggcacttgatgtaattctccttggaatttgccctttttgagtttggatcttggttcattctcaagcctcagacagtggttcaaagtttttttcttccatttcag

SEQ ID NO: 70 - DNA, 274 bp, synthetic construct
  misc_feature 1..274: note = EF-1 alpha intron fragment
  source 1..274: mol_type = other DNA
tccgtcctcagccgtcgcttcatgtgactccacggagtaccgggcgccgtccaggcacctcgattagttctcgagcttttggagtacgtcgtctttaggttggggggaggggttttatgcgatggagtttccccacactgagtgggtggagactgaagttaggccagcttggcacttgatgtaattctccttggaatttgccctttttgagtttggatcttggttcattctcaagcctcagacagtggttcaaagtttttttcttccatttcag

SEQ ID NO: 71 - DNA, 324 bp, synthetic construct
  misc_feature 1..324: note = EF-1 alpha intron fragment
  source 1..324: mol_type = other DNA
cgctcgggagagcgggcgggtgagtcacccacacaaaggaaaagggcctttccgtcctcagccgtcgcttcatgtgactccacggagtaccgggcgccgtccaggcacctcgattagttctcgagcttttggagtacgtcgtctttaggttggggggaggggttttatgcgatggagtttccccacactgagtgggtggagactgaagttaggccagcttggcacttgatgtaattctccttggaatttgccctttttgagtttggatcttggttcattctcaagcctcagacagtggttcaaagtttttttcttccatttcag

SEQ ID NO: 72 - DNA, 355 bp, synthetic construct
  misc_feature 1..355: note = EF-1 alpha intron fragment
  source 1..355: mol_type = other DNA
tgctgcagggagctcaaaatggaggacgcggcgctcgggagagcgggcgggtgagtcacccacacaaaggaaaagggcctttccgtcctcagccgtcgcttcatgtgactccacggagtaccgggcgccgtccaggcacctcgattagttctcgagcttttggagtacgtcgtctttaggttggggggaggggttttatgcgatggagtttccccacactgagtgggtggagactgaagttaggccagcttggcacttgatgtaattctccttggaatttgccctttttgagtttggatcttggttcattctcaagcctcagacagtggttcaaagtttttttcttccatttcag

SEQ ID NO: 73 - DNA, 374 bp, synthetic construct
  misc_feature 1..374: note = EF-1 alpha intron fragment
  source 1..374: mol_type = other DNA
gatggccgcttcccggccctgctgcagggagctcaaaatggaggacgcggcgctcgggagagcgggcgggtgagtcacccacacaaaggaaaagggcctttccgtcctcagccgtcgcttcatgtgactccacggagtaccgggcgccgtccaggcacctcgattagttctcgagcttttggagtacgtcgtctttaggttggggggaggggttttatgcgatggagtttccccacactgagtgggtggagactgaagttaggccagcttggcacttgatgtaattctccttggaatttgccctttttgagtttggatcttggttcattctcaagcctcagacagtggttcaaagtttttttcttccatttcag

SEQ ID NO: 74 - DNA, 424 bp, synthetic construct
  misc_feature 1..424: note = EF-1 alpha intron fragment
  source 1..424: mol_type = other DNA
gccctgggcggcaaggctggcccggtcggcaccagttgcgtgagcggaaagatggccgcttcccggccctgctgcagggagctcaaaatggaggacgcggcgctcgggagagcgggcgggtgagtcacccacacaaaggaaaagggcctttccgtcctcagccgtcgcttcatgtgactccacggagtaccgggcgccgtccaggcacctcgattagttctcgagcttttggagtacgtcgtctttaggttggggggaggggttttatgcgatggagtttccccacactgagtgggtggagactgaagttaggccagcttggcacttgatgtaattctccttggaatttgccctttttgagtttggatcttggttcattctcaagcctcagacagtggttcaaagtttttttcttccatttcag

SEQ ID NO: 75 - protein, 93 aa, synthetic construct
  REGION 1..93: note = TAFA4_Homo sapiens
IKQGTCEVVAVHRCCNKNRIEERSQTVKCSCFPGQVAGTTRAQPSCVEASIVIQKWWCHMNPCLEGEDCKVLPDYSGWSCSSGNKVKTTKVTR

SEQ ID NO: 76 - protein, 91 aa, synthetic construct
  REGION 1..91: note = TAFA1_Homo sapiens
EGGTCEVIAAHRCCNKNRIEERSQTVKCSCLPGKVAGTTRNRPSCVDASIVIGKWWCEMEPCLEGEECKTLPDNSGWMCATGNKIKTTRIH

SEQ ID NO: 77 - protein, 91 aa, synthetic construct; identical to SEQ ID NO: 76
  REGION 1..91: note = TAFA1_Macaca fascicularis_isoform1

SEQ ID NO: 78 - protein, 91 aa, synthetic construct; identical to SEQ ID NO: 76
  REGION 1..91: note = TAFA1_Sus scrofa_isoform2

SEQ ID NO: 79 - protein, 91 aa, synthetic construct; identical to SEQ ID NO: 76
  REGION 1..91: note = TAFA1_Oryctolagus cuniculus_isoform1

SEQ ID NO: 80 - protein, 91 aa, synthetic construct; identical to SEQ ID NO: 76
  REGION 1..91: note = TAFA1_Rattus norvegicus_isoform1

SEQ ID NO: 81 - protein, 91 aa, synthetic construct; identical to SEQ ID NO: 76
  REGION 1..91: note = TAFA1_Mus musculus

SEQ ID NO: 82 - protein, 91 aa, synthetic construct; identical to SEQ ID NO: 76
  REGION 1..91: note = TAFA1_Gallus gallus_isoform2

SEQ ID NO: 83 - protein, 91 aa, synthetic construct
  REGION 1..91: note = TAFA1_Varanus komodoensis
EGGTCEVIAAHRCCNKNRIEERSQTVKCSCLPGKVAGTTRNRPSCVDASIVIGKWWCEMEPCLEGEECKTLPDNSGWMCATGNKVKTTRIH

SEQ ID NO: 84 - protein, 91 aa, synthetic construct; identical to SEQ ID NO: 83
  REGION 1..91: note = TAFA1_Podarcis muralis_isoform1

SEQ ID NO: 85 - protein, 91 aa, synthetic construct; identical to SEQ ID NO: 83
  REGION 1..91: note = TAFA1_Sceloporus undulatus_isoform1

SEQ ID NO: 86 - protein, 92 aa, synthetic construct
  REGION 1..92: note = TAFA1_Xenopus tropicalis_isoform1
IEGGTCEVIAAHRCCNKNRIEERSQTVKCSCLPGKVAGTTRNRPSCVDASIVIGKWWCEMEPCLEGEECKTLPDNSGWMCATGNKIKTTRFQ

SEQ ID NO: 87 - protein, 92 aa, synthetic construct
  REGION 1..92: note = TAFA1_Xenopus tropicalis_isoform2
IEGGTCEVIAAHRCCNKNRIEERSQTVKCSCLPGKVAGTTRNRPSCVDASIVIGKWWCEMEPCLEGEECKTLPDNSGWMCATGNKIKTTRIH

SEQ ID NO: 88 - protein, 93 aa, synthetic construct
  REGION 1..93: note = TAFA1_Danio rerio_isoform1
LEGGTCEVIAAHRCCNKNKIEERSQTVKCSCLPGKVAGTTRNKPSCVDASIVIGKWWCEMEPCLEGEECKTLPDNSGWMCYSGNKIKTTRGNI

SEQ ID NO: 89 - protein, 93 aa, synthetic construct
  REGION 1..93: note = TAFA1_Danio rerio_isoform2
LEGGTCEVIAAHRCCNKNKIEERSQTVKCSCLPGKVAGTTRNKPSCVDASIVIGKWWCEMEPCLEGEECKTLPDNSGWMCYSGNKIKTTRNTH

SEQ ID NO: 90 - protein, 93 aa, synthetic construct
  REGION 1..93: note = TAFA2_Homo sapiens
VKTGTCEVVALHRCCNKNKIEERSQTVKCSCFPGQVAGTTRAAPSCVDASIVEQKWWCHMQPCLEGEECKVLPDRKGWSCSSGNKVKTTRVTH

SEQ ID NO: 91 - protein, 93 aa, synthetic construct; identical to SEQ ID NO: 90
  REGION 1..93: note = TAFA2_Macaca fascicularis

SEQ ID NO: 92 - protein, 93 aa, synthetic construct; identical to SEQ ID NO: 90
  REGION 1..93: note = TAFA2_Sus scrofa

SEQ ID NO: 93 - protein, 93 aa, synthetic construct; identical to SEQ ID NO: 90
  REGION 1..93: note = TAFA2_Oryctolagus cuniculus

SEQ ID NO: 94 - protein, 93 aa, synthetic construct
  REGION 1..93: note = TAFA2_Rattus norvegicus_isoform1
VRTGTCEVVALHRCCNKNKIEERSQTVKCSCFPGQVAGTTRAAPSCVDASIVEQKWWCHMQPCLEGEECKVLPDRKGWSCSSGNKVKTTRANV

SEQ ID NO: 95 - protein, 93 aa, synthetic construct
  REGION 1..93: note = TAFA2_Rattus norvegicus_isoform2
VRTGTCEVVALHRCCNKNKIEERSQTVKCSCFPGQVAGTTRAAPSCVDASIVEQKWWCHMQPCLEGEECKVLPDRKGWSCSSGNKVKTTRVTH

SEQ ID NO: 96 - protein, 93 aa, synthetic construct; identical to SEQ ID NO: 95
  REGION 1..93: note = TAFA2_Mus musculus_isoform1

SEQ ID NO: 97 - protein, 93 aa, synthetic construct
  REGION 1..93: note = TAFA2_Gallus gallus_isoform1
VKTGTCEVVALHRCCNKNKIEERSQTVKCSCFPGQVAGTTRAAPSCVDASIVEQKWWCHMQPCLEGEECKVLPDRKGWSCSSGNKVKTTRANV

SEQ ID NO: 98 - protein, 93 aa, synthetic construct
  REGION 1..93: note = TAFA2_Gallus gallus_isoform2
VKTGTCEVVALHRCCNKNKIEERSQTVKCSCFPGQVAGTTRAAPSCVDASIVEQKWWCHMQPCLEGEECKVLPDRKGWSCSSGNKVKTTRVTR

SEQ ID NO: 99 - protein, 93 aa, synthetic construct
  REGION 1..93: note = TAFA2_Varanus komodoensis
VKTGTCEVVALHRCCNKNKIEERSQTVKCSCFPGQVAGTTRAAPSCVDASIVEQKWWCHMQPCLEGEECKVLPDRKGWSCSSGNKVKTTRVSK

SEQ ID NO: 100 - protein, 91 aa, synthetic construct
  REGION 1..91: note = TAFA2_Podarcis muralis_isoform1
VKTGTCEVVALHRCCNKNKIEERSQTVKCSCFPGQVAGTTRAAPSCVDASIVEQKWWCHMQPCLEGEECKVLPDRKGWSCSSGNKVKTTRM

SEQ ID NO: 101 - protein, 93 aa, synthetic construct; identical to SEQ ID NO: 98
  REGION 1..93: note = TAFA2_Podarcis muralis_isoform2

SEQ ID NO: 102 - protein, 93 aa, synthetic construct; identical to SEQ ID NO: 98
  REGION 1..93: note = TAFA2_Sceloporus undulatus

SEQ ID NO: 103 - protein, 92 aa, synthetic construct
  REGION 1..92: note = TAFA2_Gekko japonicus
VKTGTCEVVALHRCCNKNKIEERSQTVKCSCFPGQVAGTTRAAPSCVDASIVEQKWWCQMQPCLEGEECKVLPDRKGWSCSSGNKVKTTRAN

SEQ ID NO: 104 - protein, 93 aa, synthetic construct
  REGION 1..93: note = TAFA2_Xenopus tropicalis
VRTGTCEVVALHRCCNKNKIEERSQTVKCSCFPGQVAGTTRATPSCVDASIVEQKWWCHMQPCLEGEECKILPDQKGWSCASGNKVKTTKVTR

SEQ ID NO: 105 - protein, 93 aa, synthetic construct
  REGION 1..93: note = TAFA2_Danio rerio
VKAGTCEVIAAHRCCNKNKIEERSQTVKCSCFPGQVAGTTRAAPSCVDASIVAQKWWCQMQPCMDGEECKVLPDLKGWSCSTGNKVKTTKVTR

SEQ ID NO: 106 - protein, 93 aa, synthetic construct
  REGION 1..93: note = TAFA3_Homo sapiens_isoform1
VQQGTCEVIAAHRCCNRNRIEERSQTVKCSCFSGQVAGTTRAKPSCVDASIVLQRWWCQMEPCLPGEECKVLPDLSGWSCSSGHKVKTTKVTR

SEQ ID NO: 107 - protein, 93 aa, synthetic construct; identical to SEQ ID NO: 106
  REGION 1..93: note = TAFA3_Macaca fascicularis_isoform3

SEQ ID NO: 108 - protein, 93 aa, synthetic construct
  REGION 1..93: note = TAFA3_Sus scrofa_isoform2
VKQGTCEVIAAHRCCNRNRIEERSQTVKCSCFSGQVAGTTRAKPSCVDASIVLQKWWCQMEPCLPGEECKVLPDLSGWSCSSGHKVKTTKVTR

SEQ ID NO: 109 - protein, 93 aa, synthetic construct
  REGION 1..93: note = TAFA3_Oryctolagus cuniculus_isoform2
VKQGTCEVIAAHRCCNQNRIEERSQTVKCSCLSGQVAGTTRAKPSCVDASIVLQRWWCQMEPCLPGEECKVLPDLSGWSCSSGHKVKTTKVTR

SEQ ID NO: 110 - protein, 93 aa, synthetic construct
  REGION 1..93: note = TAFA3_Rattus norvegicus
VKQGTCEVIAAHRCCNRNRIEERSQTVKCSCLSGQVAGTTRAKPSCVDASIVLQKWWCQMEPCLLGEECKVLPDLSGWSCSRGHKVKTTKVTR

SEQ ID NO: 111 - protein, 93 aa, synthetic construct
  REGION 1..93: note = TAFA3_Mus musculus_isoform1
VKQGTCEVIAAHRCCNRNRIEERSQTVKCSCLSGQVAGTTRAKPSCVDASIVLQKWWCQMEPCLLGEECKVLPDLSGWSCSSGHKVKTTKVTR

SEQ ID NO: 112 - protein, 93 aa, synthetic construct
  REGION 1..93: note = TAFA3_Gallus gallus
VEPGTCEVIAAHRCCNKNKIEERSQTVKCSCFPGQVAGTTRAAPSCVDASIVLQKWWCQMEPCLAGEECKVLPDLSGWSCSSGNKVKTTKVTR

SEQ ID NO: 113 - protein, 93 aa, synthetic construct
  REGION 1..93: note = TAFA3_Varanus komodoensis_isoform2
IEPGTCEVIAAHRCCNKNKIEERSQTVKCSCFPGQVAGTTRAAPSCVDASIVLQKWWCQMQPCLEGEECKVLPDLSGWSCSTGNKVKTTKVTR

SEQ ID NO: 114 - protein, 93 aa, synthetic construct
  REGION 1..93: note = TAFA3_Podarcis muralis
IEPGTCEVIAAHRCCNKNKIEERSQTVKCSCFPGQVAGTTHAAPSCVDASIVLQKWWCQMQPCVEGEECKVLPDLSGWSCSTGNKVKTTKVTR

SEQ ID NO: 115 - protein, 93 aa, synthetic construct; identical to SEQ ID NO: 113
  REGION 1..93: note = TAFA3_Sceloporus undulatus

SEQ ID NO: 116 - protein, 93 aa, synthetic construct
  REGION 1..93: note = TAFA3_Xenopus tropicalis_isoform2
VEPGTCEVIAAHRCCNKNKIEERSQTVKCSCFPGQVAGTTRAAPSCVDASIVIQKWWCQMEPCLEGEDCKVLPDLSGWSCSTGNKVKTTKVTR

SEQ ID NO: 117 - protein, 93 aa, synthetic construct
  REGION 1..93: note = TAFA3_Danio rerio
VKAGTCEVIAAHRCCNRNKIEERSQTVKCSCFPGQVAGTTRAAPSCVDASIVAQKWWCQMQPCVDGEECKVLPDLTGWSCSTGNKVKTTKVTR

SEQ ID NO: 118 - protein, 93 aa, synthetic construct; identical to SEQ ID NO: 75
  REGION 1..93: note = TAFA4_Macaca fascicularis_isoform2

SEQ ID NO: 119 - protein, 93 aa, synthetic construct; identical to SEQ ID NO: 75
  REGION 1..93: note = TAFA4_Sus scrofa_isoform2

SEQ ID NO: 120 - protein, 93 aa, synthetic construct
  REGION 1..93: note = TAFA4_Oryctolagus cuniculus_isoform4
IKPGTCEVVAVHRCCNKNRIEERSQTVKCSCFPGQVAGTTQAQPSCVEASIVAQKWWCHMNPCLEGEDCKVLPDYSGWSCSSGNKVKTTKVTR

SEQ ID NO: 121 - protein, 93 aa, synthetic construct
  REGION 1..93: note = TAFA4_Rattus norvegicus
IKQGTCEVVAVHRCCNKNRIEERSQTVKCSCFPGQVAGTTRAQPSCVEASIVIEKWWCHMDPCLEGEDCKVLPDSSGWSCSSGNKVKTTKVTR

SEQ ID NO: 122 - protein, 93 aa, synthetic construct
  REGION 1..93: note = TAFA4_Mus musculus
IKPGTCEVVAVHRCCNKNRIEERSQTVKCSCFPGQVAGTTRAQPSCVEAAIVIEKWWCHMNPCLEGEDCKVLPDSSGWSCSSGNKVKTTKVTR

SEQ ID NO: 123 - protein, 93 aa, synthetic construct
  REGION 1..93: note = TAFA4_Gallus gallus
VKQGTCEVVAVHRCCNKNRIEERSQTVKCSCFPGQVAGTTRAQPSCVEASIVLQKWWCHMNPCLDGEDCKVLPDYSGWSCSSGNKVKTTKVTR

SEQ ID NO: 124 - protein, 93 aa, synthetic construct
  REGION 1..93: note = TAFA4_Varanus komodoensis_isoform2
VKQGTCEVVAVHRCCNKNRIEERSQTVKCSCLPGQVAGTTRAQPSCVEAAIVVQKWWCHMNPCLEGEECKVLPDYSGWSCSSGNKVKTTKVTR

SEQ ID NO: 125 - protein, 93 aa, synthetic construct
  REGION 1..93: note = TAFA4_Podarcis muralis
VKQGTCEVVAVHRCCNKNRIEERSQTVKCSCFPGQVAGTTRAQPSCVEAAIVIQKWWCHMNPCLDGEDCKVLPDYSGWSCSSGNKVKTTKVTR

SEQ ID NO: 126 - protein, 93 aa, synthetic construct
  REGION 1..93: note = TAFA4_Sceloporus undulatus
VKQGTCEVVAVHRCCNKNRIEERSQTVKCSCFPGQVAGTTRSQPSCVEAAIVIQKWWCHMNPCLEGEECKVLPDYSGWSCSSGNKVKTTKVTR

SEQ ID NO: 127 - protein, 93 aa, synthetic construct
  REGION 1..93: note = TAFA4_Gekko japonicus
VKQGTCEVVAVHLCCNKNRIEELSQTGNCSCLPGQVAGTTRTQPSCVEAAIVIQKWWCQMSPCLEGEECKVLPDSSGWSCSSGNKVKTTKVTR

SEQ ID NO: 128 - protein, 93 aa, synthetic construct
  REGION 1..93: note = TAFA4_Xenopus tropicalis
VKQGTCEVVALHRCCNKNRIEERSQTVKCSCFPGQVAGTTRAQPSCVEASIVIQKWWCHMNPCMEGEECKVLPDLTGWSCSSGNKIKTTKVTR

SEQ ID NO: 129 - protein, 93 aa, synthetic construct
  REGION 1..93: note = TAFA4_Danio rerio
VKQGTCEVVAIHRCCNKNKIEERSQTVKCSCFPGQVAGTTRAQPSCVEASIVLQKWWCQMHPCLDGEECKALPDLTGWSCSTGNKVKTTKVTR

SEQ ID NO: 130 - protein, 98 aa, synthetic construct
  REGION 1..98: note = TAFA1_Homo sapiens
LHRPEGGTCEVIAAHRCCNKNRIEERSQTVKCSCLPGKVAGTTRNRPSCVDASIVIGKWWCEMEPCLEGEECKTLPDNSGWMCATGNKIKTTRIHPRT

SEQ ID NO: 131 - protein, 98 aa, synthetic construct; identical to SEQ ID NO: 130
  REGION 1..98: note = TAFA1_Macaca fascicularis_isoform1

SEQ ID NO: 132 - protein, 98 aa, synthetic construct; identical to SEQ ID NO: 130
  REGION 1..98: note = TAFA1_Sus scrofa_isoform2

SEQ ID NO: 133 - protein, 98 aa, synthetic construct; identical to SEQ ID NO: 130
  REGION 1..98: note = TAFA1_Oryctolagus cuniculus_isoform1

SEQ ID NO: 134 - protein, 98 aa, synthetic construct; identical to SEQ ID NO: 130
  REGION 1..98: note = TAFA1_Rattus norvegicus_isoform1

SEQ ID NO: 135 - protein, 98 aa, synthetic construct; identical to SEQ ID NO: 130
  REGION 1..98: note = TAFA1_Mus musculus

SEQ ID NO: 136 - protein, 98 aa, synthetic construct; identical to SEQ ID NO: 130
  REGION 1..98: note = TAFA1_Gallus gallus_isoform2

SEQ ID NO: 137 - protein, 98 aa, synthetic construct
  REGION 1..98: note = TAFA1_Varanus komodoensis
LHRPEGGTCEVIAAHRCCNKNRIEERSQTVKCSCLPGKVAGTTRNRPSCVDASIVIGKWWCEMEPCLEGEECKTLPDNSGWMCATGNKVKTTRIHPRT

SEQ ID NO: 138 - protein, 98 aa, synthetic construct; identical to SEQ ID NO: 137
  REGION 1..98: note = TAFA1_Podarcis muralis_isoform1

SEQ ID NO: 139 - protein, 98 aa, synthetic construct; identical to SEQ ID NO: 137
  REGION 1..98: note = TAFA1_Sceloporus undulatus_isoform1

SEQ ID NO: 140 - protein, 114 aa, synthetic construct
  REGION 1..114: note = TAFA1_Xenopus tropicalis_isoform1
LHQSGFTSGHFPHHRKLGEIEGGTCEVIAAHRCCNKNRIEERSQTVKCSCLPGKVAGTTRNRPSCVDASIVIGKWWCEMEPCLEGEECKTLPDNSGWMCATGNKIKTTRFQGHL

SEQ ID NO: 141 - protein, 114 aa, synthetic construct
  REGION 1..114: note = TAFA1_Xenopus tropicalis_isoform2
LHQSGFTSGHFPHHRKLGEIEGGTCEVIAAHRCCNKNRIEERSQTVKCSCLPGKVAGTTRNRPSCVDASIVIGKWWCEMEPCLEGEECKTLPDNSGWMCATGNKIKTTRIHPRS

SEQ ID NO: 142 - protein, 109 aa, synthetic construct
  REGION 1..109: note = TAFA1_Danio rerio_isoform1
LAPPGTNIQILEGGTCEVIAAHRCCNKNKIEERSQTVKCSCLPGKVAGTTRNKPSCVDASIVIGKWWCEMEPCLEGEECKTLPDNSGWMCYSGNKIKTTRGNIQEDKLK

SEQ ID NO: 143 - protein, 108 aa, synthetic construct
  REGION 1..108: note = TAFA1_Danio rerio_isoform2
LAPPGTNIQILEGGTCEVIAAHRCCNKNKIEERSQTVKCSCLPGKVAGTTRNKPSCVDASIVIGKWWCEMEPCLEGEECKTLPDNSGWMCYSGNKIKTTRNTHPYTSL

SEQ ID NO: 144 - protein, 101 aa, synthetic construct
  REGION 1..101: note = TAFA2_Homo sapiens
ANHHKAHHVKTGTCEVVALHRCCNKNKIEERSQTVKCSCFPGQVAGTTRAAPSCVDASIVEQKWWCHMQPCLEGEECKVLPDRKGWSCSSGNKVKTTRVTH

SEQ ID NO: 145 - protein, 101 aa, synthetic construct; identical to SEQ ID NO: 144
  REGION 1..101: note = TAFA2_Macaca fascicularis

SEQ ID NO: 146 - protein, 101 aa, synthetic construct
  REGION 1..101: note = TAFA2_Sus scrofa
VNHHKAHHVKTGTCEVVALHRCCNKNKIEERSQTVKCSCFPGQVAGTTRAAPSCVDASIVEQKWWCHMQPCLEGEECKVLPDRKGWSCSSGNKVKTTRVTH

SEQ ID NO: 147 - protein, 101 aa, synthetic construct; identical to SEQ ID NO: 144
  REGION 1..101: note = TAFA2_Oryctolagus cuniculus

SEQ ID NO: 148 - protein, 101 aa, synthetic construct
  REGION 1..101: note = TAFA2_Rattus norvegicus_isoform1
ANHHKAHHVRTGTCEVVALHRCCNKNKIEERSQTVKCSCFPGQVAGTTRAAPSCVDASIVEQKWWCHMQPCLEGEECKVLPDRKGWSCSSGNKVKTTRANV

SEQ ID NO: 149 - protein, 101 aa, synthetic construct
  REGION 1..101: note = TAFA2_Rattus norvegicus_isoform2
ANHHKAHHVRTGTCEVVALHRCCNKNKIEERSQTVKCSCFPGQVAGTTRAAPSCVDASIVEQKWWCHMQPCLEGEECKVLPDRKGWSCSSGNKVKTTRVTH

SEQ ID NO: 150 - protein, 101 aa, synthetic construct; identical to SEQ ID NO: 149
  REGION 1..101: note = TAFA2_Mus musculus_isoform1

SEQ ID NO: 151 - protein, 101 aa, synthetic construct
  REGION 1..101: note = TAFA2_Gallus gallus_isoform1
ANHHKAHHVKTGTCEVVALHRCCNKNKIEERSQTVKCSCFPGQVAGTTRAAPSCVDASIVEQKWWCHMQPCLEGEECKVLPDRKGWSCSSGNKVKTTRANV

SEQ ID NO: 152 - protein, 101 aa, synthetic construct
  REGION 1..101: note = TAFA2_Gallus gallus_isoform2
ANHHKAHHVKTGTCEVVALHRCCNKNKIEERSQTVKCSCFPGQVAGTTRAAPSCVDASIVEQKWWCHMQPCLEGEECKVLPDRKGWSCSSGNKVKTTRVTR

SEQ ID NO: 153 - protein, 119 aa, synthetic construct
  REGION 1..119: note = TAFA2_Varanus komodoensis
ANHHKAHHVKTGTCEVVALHRCCNKNKIEERSQTVKCSCFPGQVAGTTRAAPSCVDASIVEQKWWCHMQPCLEGEECKVLPDRKGWSCSSGNKVKTTRVSKRVKPFKNKEISAVPDDNF

SEQ ID NO: 154 - protein, 106 aa, synthetic construct
  REGION 1..106: note = TAFA2_Podarcis muralis_isoform1
ANHHKAHHVKTGTCEVVALHRCCNKNKIEERSQTVKCSCFPGQVAGTTRAAPSCVDASIVEQKWWCHMQPCLEGEECKVLPDRKGWSCSSGNKVKTTRMFWCCATE

SEQ ID NO: 155 - protein, 101 aa, synthetic construct; identical to SEQ ID NO: 152
  REGION 1..101: note = TAFA2_Podarcis muralis_isoform2

SEQ ID NO: 156 - protein, 101 aa, synthetic construct; identical to SEQ ID NO: 152
  REGION 1..101: note = TAFA2_Sceloporus undulatus

SEQ ID NO: 157 - protein, 101 aa, synthetic construct
  REGION 1..101: note = TAFA2_Gekko japonicus
ANHHKAHHVKTGTCEVVALHRCCNKNKIEERSQTVKCSCFPGQVAGTTRAAPSCVDASIVEQKWWCQMQPCLEGEECKVLPDRKGWSCSSGNKVKTTRANV

SEQ ID NO: 158 - protein, 101 aa, synthetic construct
  REGION 1..101: note = TAFA2_Xenopus tropicalis
VIHHKAQHVRTGTCEVVALHRCCNKNKIEERSQTVKCSCFPGQVAGTTRATPSCVDASIVEQKWWCHMQPCLEGEECKILPDQKGWSCASGNKVKTTKVTR

SEQ ID NO: 159 - protein, 103 aa, synthetic construct
  REGION 1..103: note = TAFA3_Homo sapiens_isoform1
ALQPPTATVLVQQGTCEVIAAHRCCNRNRIEERSQTVKCSCFSGQVAGTTRAKPSCVDASIVLQRWWCQMEPCLPGEECKVLPDLSGWSCSSGHKVKTTKVTR

SEQ ID NO: 160 - protein, 103 aa, synthetic construct; identical to SEQ ID NO: 159
  REGION 1..103: note = TAFA3_Macaca fascicularis_isoform3

SEQ ID NO: 161 - protein, 103 aa, synthetic construct
  REGION 1..103: note = TAFA3_Sus scrofa_isoform2
SLQLPTPTVLVKQGTCEVIAAHRCCNRNRIEERSQTVKCSCFSGQVAGTTRAKPSCVDASIVLQKWWCQMEPCLPGEECKVLPDLSGWSCSSGHKVKTTKVTR

SEQ ID NO: 162 - protein, 103 aa, synthetic construct
  REGION 1..103: note = TAFA3_Oryctolagus cuniculus_isoform2
SLEPPTTAVLVKQGTCEVIAAHRCCNQNRIEERSQTVKCSCLSGQVAGTTRAKPSCVDASIVLQRWWCQMEPCLPGEECKVLPDLSGWSCSSGHKVKTTKVTR

SEQ ID NO: 163 - protein, 103 aa, synthetic construct
  REGION 1..103: note = TAFA3_Rattus norvegicus
SLQPPTSTVLVKQGTCEVIAAHRCCNRNRIEERSQTVKCSCLSGQVAGTTRAKPSCVDASIVLQKWWCQMEPCLLGEECKVLPDLSGWSCSRGHKVKTTKVTR

SEQ ID NO: 164 - protein, 103 aa, synthetic construct
  REGION 1..103: note = TAFA3_Mus musculus_isoform1
SLQPPTSAVLVKQGTCEVIAAHRCCNRNRIEERSQTVKCSCLSGQVAGTTRAKPSCVDASIVLQKWWCQMEPCLLGEECKVLPDLSGWSCSSGHKVKTTKVTR

SEQ ID NO: 165 - protein, 103 aa, synthetic construct
  REGION 1..103: note = TAFA3_Gallus gallus
STHHRSHSAHVEPGTCEVIAAHRCCNKNKIEERSQTVKCSCFPGQVAGTTRAAPSCVDASIVLQKWWCQMEPCLAGEECKVLPDLSGWSCSSGNKVKTTKVTR

SEQ ID NO: 166 - protein, 103 aa, synthetic construct
  REGION 1..103: note = TAFA3_Varanus komodoensis_isoform2
SSHHRSHSVHIEPGTCEVIAAHRCCNKNKIEERSQTVKCSCFPGQVAGTTRAAPSCVDASIVLQKWWCQMQPCLEGEECKVLPDLSGWSCSTGNKVKTTKVTR

SEQ ID NO: 167 - protein, 103 aa, synthetic construct
  REGION 1..103: note = TAFA3_Podarcis muralis
SSHHRSHSVHIEPGTCEVIAAHRCCNKNKIEERSQTVKCSCFPGQVAGTTHAAPSCVDASIVLQKWWCQMQPCVEGEECKVLPDLSGWSCSTGNKVKTTKVTR

SEQ ID NO: 168 - protein, 103 aa, synthetic construct; identical to SEQ ID NO: 166
  REGION 1..103: note = TAFA3_Sceloporus undulatus

SEQ ID NO: 169 - protein, 103 aa, synthetic construct
  REGION 1..103: note = TAFA3_Xenopus tropicalis_isoform2
SSHHRIHSVHVEPGTCEVIAAHRCCNKNKIEERSQTVKCSCFPGQVAGTTRAAPSCVDASIVIQKWWCQMEPCLEGEDCKVLPDLSGWSCSTGNKVKTTKVTR

SEQ ID NO: 170 - protein, 102 aa, synthetic construct
  REGION 1..102: note = TAFA3_Danio rerio
SSHRSHIVHVKAGTCEVIAAHRCCNRNKIEERSQTVKCSCFPGQVAGTTRAAPSCVDASIVAQKWWCQMQPCVDGEECKVLPDLTGWSCSTGNKVKTTKVTR

SEQ ID NO: 171 - protein, 95 aa, synthetic construct
  REGION 1..95: note = TAFA4_Homo sapiens
HQIKQGTCEVVAVHRCCNKNRIEERSQTVKCSCFPGQVAGTTRAQPSCVEASIVIQKWWCHMNPCLEGEDCKVLPDYSGWSCSSGNKVKTTKVTR

SEQ ID NO: 172 - protein, 95 aa, synthetic construct; identical to SEQ ID NO: 171
  REGION 1..95: note = TAFA4_Macaca fascicularis_isoform2

SEQ ID NO: 173 - protein, 95 aa, synthetic construct; identical to SEQ ID NO: 171
  REGION 1..95: note = TAFA4_Sus scrofa_isoform2

SEQ ID NO: 174 - protein, 95 aa, synthetic construct
  REGION 1..95: note = TAFA4_Oryctolagus cuniculus_isoform4
HQIKPGTCEVVAVHRCCNKNRIEERSQTVKCSCFPGQVAGTTQAQPSCVEASIVAQKWWCHMNPCLEGEDCKVLPDYSGWSCSSGNKVKTTKVTR

SEQ ID NO: 175 - protein, 95 aa, synthetic construct
  REGION 1..95: note = TAFA4_Rattus norvegicus
HVIKQGTCEVVAVHRCCNKNRIEERSQTVKCSCFPGQVAGTTRAQPSCVEASIVIEKWWCHMDPCLEGEDCKVLPDSSGWSCSSGNKVKTTKVTR

SEQ ID NO: 176 - protein, 95 aa, synthetic construct
  REGION 1..95: note = TAFA4_Mus musculus
HLIKPGTCEVVAVHRCCNKNRIEERSQTVKCSCFPGQVAGTTRAQPSCVEAAIVIEKWWCHMNPCLEGEDCKVLPDSSGWSCSSGNKVKTTKVTR

SEQ ID NO: 177 - protein, 95 aa, synthetic construct
  REGION 1..95: note = TAFA4_Gallus gallus
HQVKQGTCEVVAVHRCCNKNRIEERSQTVKCSCFPGQVAGTTRAQPSCVEASIVLQKWWCHMNPCLDGEDCKVLPDYSGWSCSSGNKVKTTKVTR

SEQ ID NO: 178 - protein, 95 aa, synthetic construct
  REGION 1..95: note = TAFA4_Varanus komodoensis_isoform2
HQVKQGTCEVVAVHRCCNKNRIEERSQTVKCSCLPGQVAGTTRAQPSCVEAAIVVQKWWCHMNPCLEGEECKVLPDYSGWSCSSGNKVKTTKVTR

SEQ ID NO: 179 - protein, 95 aa, synthetic construct
  REGION 1..95: note = TAFA4_Podarcis muralis
HQVKQGTCEVVAVHRCCNKNRIEERSQTVKCSCFPGQVAGTTRAQPSCVEAAIVIQKWWCHMNPCLDGEDCKVLPDYSGWSCSSGNKVKTTKVTR

SEQ ID NO: 180 - protein, 95 aa, synthetic construct
  REGION 1..95: note = TAFA4_Sceloporus undulatus
HQVKQGTCEVVAVHRCCNKNRIEERSQTVKCSCFPGQVAGTTRSQPSCVEAAIVIQKWWCHMNPCLEGEECKVLPDYSGWSCSSGNKVKTTKVTR

SEQ ID NO: 181 - protein, 95 aa, synthetic construct
  REGION 1..95: note = TAFA4_Gekko japonicus
HQVKQGTCEVVAVHLCCNKNRIEELSQTGNCSCLPGQVAGTTRTQPSCVEAAIVIQKWWCQMSPCLEGEECKVLPDSSGWSCSSGNKVKTTKVTR

SEQ ID NO: 182 - protein, 95 aa, synthetic construct
  REGION 1..95: note = TAFA4_Xenopus tropicalis
YQVKQGTCEVVALHRCCNKNRIEERSQTVKCSCFPGQVAGTTRAQPSCVEASIVIQKWWCHMNPCMEGEECKVLPDLTGWSCSSGNKIKTTKVTR

SEQ ID NO: 183 - protein, 95 aa, synthetic construct
  REGION 1..95: note = TAFA4_Danio rerio
YQVKQGTCEVVAIHRCCNKNKIEERSQTVKCSCFPGQVAGTTRAQPSCVEASIVLQKWWCQMHPCLDGEECKALPDLTGWSCSTGNKVKTTKVTR

SEQ ID NO: 184 - DNA, 279 bp, synthetic construct
  misc_feature 1..279: note = TAFA4_Homo sapiens
  source 1..279: mol_type = other DNA
atcaagcaagggacctgtgaggtggtcgccgtgcacaggtgctgcaataagaaccgcatagaagagcggtcacaaacggtcaagtgctcttgcttcccgggacaggtggcgggcacaactcgggctcaaccttcttgtgttgaagcttccattgtgattcagaaatggtggtgtcacatgaatccgtgtttggaaggagaggattgtaaagtgctgccagattactcaggttggtcctgtagcagtggcaataaagtcaaaactacgaaggtaacgcgg

SEQ ID NO: 185 - DNA, 273 bp, synthetic construct
  misc_feature 1..273: note = TAFA1_Homo sapiens
  source 1..273: mol_type = other DNA
gaaggagggacgtgtgaagtgatagcagcacaccgatgttgtaacaagaatcgcattgaggagcggtcacaaacagtaaagtgttcctgtctacctggaaaagtggctggaacaacaagaaaccggccttcttgcgtcgatgcctccatagtgattgggaaatggtggtgtgagatggagccttgcctagaaggagaagaatgtaagacactccctgacaattctggatggatgtgcgcaacaggcaacaaaattaagaccacgagaattcac

SEQ ID NO: 186 - DNA, 273 bp, synthetic construct
  misc_feature 1..273: note = TAFA1_Macaca fascicularis_isoform1
  source 1..273: mol_type = other DNA
gaaggagggacgtgtgaagtgatagcagcacaccgatgttgtaacaagaatcgcattgaggagaggtcacaaacagtaaagtgttcctgtctacctggaaaagtggctggaacaacaagaaaccggccttcctgtgttgacgcctccatagtgattgggaaatggtggtgtgagatggagccttgcctagaaggagaagaatgtaagacactccctgacaattctggatggatgtgcgcaacaggcaacaaaattaagaccacgagaattcac

SEQ ID NO: 187 - DNA, 273 bp, synthetic construct
  misc_feature 1..273: note = TAFA1_Sus scrofa_isoform2
  source 1..273: mol_type = other DNA
gaaggagggacatgtgaagtgattgccgcacacagatgttgtaataagaatcgcattgaggagcggtcacaaacagtcaagtgttcctgtctacctgggaaagtggctggaacaacaagaaaccgaccttcctgtgttgatgcctccatagtgattgggaaatggtggtgtgagatggagccttgtctagaaggagaagaatgcaaaacactccctgataattctggatggatgtgtgctacaggcaataaaattaagaccacaagaattcac

SEQ ID NO: 188 - DNA, 273 bp, synthetic construct
  misc_feature 1..273: note = TAFA1_Oryctolagus cuniculus_isoform1
  source 1..273: mol_type = other DNA
gaaggagggacatgcgaggtgatagcagcacacagatgttgtaacaagaaccgcattgaggagcggtcgcaaacggtgaagtgttcctgtctccctgggaaagtggcaggaaccacaagaaaccgaccttcctgtgtggatgcctccattgtgattgggaaatggtggtgtgagatggagccttgtctagagggagaagaatgtaagacactccctgacaattctggatggatgtgcgcgacaggcaacaaaattaagaccacacgaatccat

SEQ ID NO: 189 - DNA, 273 bp, synthetic construct
  misc_feature 1..273: note = TAFA1_Rattus norvegicus_isoform1
  source 1..273: mol_type = other DNA
gaaggagggacctgtgaagtgatagcggcccacaggtgttgcaacaagaaccgcattgaggagcggtcacaaacagtgaagtgttcctgtctacctgggaaagtggctgggacaacaagaaaccgaccttcctgtgttgatgcctccatagtgattgggaaatggtggtgtgagatggaaccctgcctagaaggagaagaatgtaagacactccctgacaactctggatggatgtgtgctacaggcaacaagatcaagaccacacgaattcac

SEQ ID NO: 190 - DNA, 273 bp, synthetic construct
  misc_feature 1..273: note = TAFA1_Mus musculus
  source 1..273: mol_type = other DNA
gaaggagggacctgtgaagtgatcgcggcccacaggtgttgtaacaagaaccgcatcgaggagcggtcacaaacagtgaagtgttcctgtttacctgggaaagtggctgggacaacaagaaaccgaccttcctgtgtggatgcctccatagtaattgggaaatggtggtgtgagatggagccctgcctagaaggagaagaatgtaagacactccctgacaattctggatggatgtgtgctacaggcaacaagattaagactacacgaattcac

SEQ ID NO: 191 - DNA, 273 bp, synthetic construct
  misc_feature 1..273: note = TAFA1_Gallus gallus_isoform2
  source 1..273: mol_type = other DNA
gaaggaggaacgtgtgaagttatagcagcacacagatgctgtaataagaatcgaattgaggaaagatcacaaacagtaaaatgctcctgtctacctgggaaagtggctgggactacacgaaacagaccttcctgtgttgatgcttcaatagtgattgggaaatggtggtgtgagatggagccctgcctagaaggagaggaatgtaagacgttgcctgataattctggatggatgtgtgcgactggcaataaaatcaagaccaccagaatccac

SEQ ID NO: 192 - DNA, 273 bp, synthetic construct
  misc_feature 1..273: note = TAFA1_Varanus komodoensis
  source 1..273: mol_type = other DNA
gaagggggaacgtgtgaagttatagctgcacacagatgctgcaacaagaatcggattgaggagagatcacaaacagtaaagtgctcctgtctacctgggaaagtggctgggacaacgcggaacagaccatcatgtgttgacgcatcaatagtcattgggaaatggtggtgtgaaatggagccctgcctagagggtgaggaatgcaagacattgccggacaattcaggatggatgtgcgcaaccggcaataaagtcaagaccaccagaattcac

SEQ ID NO: 193 - DNA, 273 bp, synthetic construct
  misc_feature 1..273: note = TAFA1_Podarcis muralis_isoform1
  source 1..273: mol_type = other DNA
gaaggagggacgtgtgaagttatagcagcacacagatgttgtaataagaatcggattgaagagagatcacaaacagtaaaatgctcctgtctacctgggaaagtggccgggacgacgcggaacagaccgtcgtgtgttgatgcatcaatagtcattgggaaatggtggtgtgagatggagccatgcctagagggcgaggaatgcaagacgttacctgacaactcaggatggatgtgtgcaaccggcaataaagtcaagaccaccagaattcat

SEQ ID NO: 194 - DNA, 273 bp, synthetic construct
  misc_feature 1..273: note = TAFA1_Sceloporus undulatus_isoform1
  source 1..273: mol_type = other DNA
gaaggaggcacgtgtgaagttatagcagcacatagatgttgtaataagaatcggattgaggagagatcacaaacagtaaagtgctcctgtctacctggaaaagtggctggcacgacgcggaacagaccatcatgtgttgacgcgtccatagttattgggaaatggtggtgtgaaatggagccctgcctagagggtgaagaatgcaaaacattacctgacaattcaggatggatgtgtgcaactggcaataaagtcaagaccaccagaattcac

SEQ ID NO: 195 - DNA, 276 bp, synthetic construct
  misc_feature 1..276: note = TAFA1_Xenopus tropicalis_isoform1
  source 1..276: mol_type = other DNA
atagaaggtggaacctgtgaagttatagctgcgcacagatgctgcaataagaatcgcatcgaggaacgctcacagaccgtgaaatgttcttgtcttcctggaaaagtggctggaacgacacggaacaggccctcttgtgtcgatgcttccatagttattggaaaatggtggtgtgagatggaaccttgtttagaaggggaagaatgtaagacccttcccgacaactcgggctggatgtgtgccaccggcaataagatcaagaccacaagatttcag

SEQ ID NO: 196 - DNA, 276 bp, synthetic construct
  misc_feature 1..276: note = TAFA1_Xenopus tropicalis_isoform2
  source 1..276: mol_type = other DNA
atagaaggtggaacctgtgaagttatagctgcgcacagatgctgcaataagaatcgcatcgaggaacgctcacagaccgtgaaatgttcttgtcttcctggaaaagtggctggaacgacacggaacaggccctcttgtgtcgatgcttccatagttattggaaaatggtggtgtgagatggaaccttgtttagaaggggaagaatgtaagacccttcccgacaactcgggctggatgtgtgccaccggcaataagatcaagaccacaagaattcac

SEQ ID NO: 197 - DNA, 279 bp, synthetic construct
  misc_feature 1..279: note = TAFA1_Danio rerio_isoform1
  source 1..279: mol_type = other DNA
ctcgaaggagggacatgcgaggtgatcgcggcgcacaggtgctgtaacaaaaacaagattgaagagagatctcagacagtgaagtgctcctgtttacctgggaaagtggcaggaaccaccaggaacaaaccctcctgtgttgacgcctccattgtgattgggaagtggtggtgtgagatggagccgtgtctggagggagaagagtgtaagactctaccagacaactccggctggatgtgctactctggaaacaagatcaaaaccaccaggggaaacatc

SEQ ID NO: 198 - DNA, 279 bp, synthetic construct
  misc_feature 1..279: note = TAFA1_Danio rerio_isoform2
  source 1..279: mol_type = other DNA
ctcgaaggagggacatgcgaggtgatcgcggcgcacaggtgctgtaacaaaaacaagattgaagagagatctcagacagtgaagtgctcctgtttacctgggaaagtggcaggaaccaccaggaacaaaccctcctgtgttgacgcctccattgtgattgggaagtggtggtgtgagatggagccgtgtctggagggagaagagtgtaagactctaccagacaactccggctggatgtgctactctggaaacaagatcaaaaccaccaggaatacccac

SEQ ID NO: 199 - DNA, 279 bp, synthetic construct
  misc_feature 1..279: note = TAFA2_Homo sapiens
  source 1..279: mol_type = other DNA
gttaaaacgggaacttgtgaggtggtggcactccacagatgctgtaataagaacaagatagaagaacggtcacaaacagtcaagtgctcctgcttccctgggcaggtggcaggcaccacgcgagctgctccatcatgtgtggatgcttcaatagtggaacagaaatggtggtgccatatgcagccatgtctagagggagaagaatgtaaagttcttccggatcggaaaggatggagctgttcctctgggaataaagtcaaaacaactagggtaacccat

SEQ ID NO: 200 - DNA, 279 bp, synthetic construct
  misc_feature 1..279: note = TAFA2_Macaca fascicularis
  source 1..279: mol_type = other DNA
gttaaaacgggaacttgtgaggtggtggcactccacagatgctgtaataagaacaagatagaagaacggtcacaaacagtcaagtgctcctgcttccccgggcaggtggcaggcaccacgcgagctgctccatcatgtgtggatgcttcaatagtggaacagaaatggtggtgccatatgcagccatgtctagagggagaagaatgtaaagttcttccagatcggaaaggatggagctgttcctctgggaataaagtcaaaacaactagggtaacccat

SEQ ID NO: 201 - DNA, 279 bp, synthetic construct
  misc_feature 1..279: note = TAFA2_Sus scrofa
  source 1..279: mol_type = other DNA
gttaaaacgggcacttgtgaggtggtggcactccacagatgctgtaataagaacaagatagaagaacggtcacaaacagtcaagtgctcctgcttccctgggcaggtggcaggcaccacacgggctgctccatcttgtgtggatgcttcaatagtggaacagaaatggtggtgccatatgcaaccgtgtcttgagggagaggaatgtaaagttcttccagatcggaaaggatggagctgttcctctgggaataaagtgaaaacaacaagggtaacccat

SEQ ID NO: 202 - DNA, 279 bp, synthetic construct
  misc_feature 1..279: note = TAFA2_Oryctolagus cuniculus
  source 1..279: mol_type = other DNA
gttaaaacgggaacttgtgaggtggtggcactccacagatgctgtaataagaacaagatagaagaacggtcacaaactgtcaaatgctcctgcttcccggggcaggtggccggcaccacgcgagctgctccatcttgtgtggatgcttcaatagtagagcagaaatggtggtgccatatgcagccatgtctagagggagaagaatgtaaagttcttcctgatcggaaaggatggagctgttcctctgggaataaagtgaaaactactagagtaacccat

SEQ ID NO: 203 - DNA, 279 bp, synthetic construct
  misc_feature 1..279: note = TAFA2_Rattus norvegicus_isoform1
  source 1..279: mol_type = other DNA
gttagaactgggacttgcgaggtggtggcgctgcacagatgctgtaataagaacaagatagaagaacggtcccaaacggtcaagtgctcctgcttccctgggcaggtggcaggcactacccgagctgccccatcttgtgtggatgcatccatagtggaacaaaaatggtggtgtcatatgcagccatgtctggagggagaggaatgtaaagtccttccagatcgcaaaggatggagctgttcctctggaaacaaagtaaaaacaactagggcaaacgtg

SEQ ID NO: 204 - DNA, 279 bp, synthetic construct
  misc_feature 1..279: note = TAFA2_Rattus norvegicus_isoform2
  source 1..279: mol_type = other DNA
gttagaactgggacttgcgaggtggtggcgctgcacagatgctgtaataagaacaagatagaagaacggtcccaaacggtcaagtgctcctgcttccctgggcaggtggcaggcactacccgagctgccccatcttgtgtggatgcatccatagtggaacaaaaatggtggtgtcatatgcagccatgtctggagggagaggaatgtaaagtccttccagatcgcaaaggatggagctgttcctctggaaacaaagtaaaaacaactagggtaactcat

SEQ ID NO: 205 - DNA, 279 bp, synthetic construct
  misc_feature 1..279: note = TAFA2_Mus musculus_isoform1
  source 1..279: mol_type = other DNA
gttagaactgggacttgcgaggttgtggcgctgcacagatgctgtaataagaacaagatagaagaacggtcccaaacggtcaagtgctcctgcttccctgggcaggtggcaggcactacccgagctgctccgtcttgtgtggatgcatccatagtggaacaaaagtggtggtgtcatatgcagccatgcctggagggagaggaatgtaaagtccttccagatcgcaaaggatggagctgttcctctggaaacaaagtaaaaacaactagggtaacccat

SEQ ID NO: 206 - DNA, 279 bp, synthetic construct
  misc_feature 1..279: note = TAFA2_Gallus gallus_isoform1
  source 1..279: mol_type = other DNA
gttaaaactgggacctgtgaagtggtggcactccacagatgttgcaataagaacaagatagaagaaagatcacagacagtgaagtgctcctgcttccctgggcaggtagcaggtaccactcgggcagctccttcttgtgttgatgcttcaatagtggagcagaaatggtggtgccacatgcaaccatgtcttgaaggggaggaatgtaaggttcttccagatcgtaagggatggagctgttcctccgggaataaagtgaaaacaactagggcaaacgtg

SEQ ID NO: 207 - DNA, 279 bp, synthetic construct
  misc_feature 1..279: note = TAFA2_Gallus gallus_isoform2
  source 1..279: mol_type = other DNA
gttaaaactgggacctgtgaagtggtggcactccacagatgttgcaataagaacaagatagaagaaagatcacagacagtgaagtgctcctgcttccctgggcaggtagcaggtaccactcgggcagctccttcttgtgttgatgcttcaatagtggagcagaaatggtggtgccacatgcaaccatgtcttgaaggggaggaatgtaaggttcttccagatcgtaagggatggagctgttcctccgggaataaagtgaaaacaactagggtaacccga

SEQ ID NO: 208 - DNA, 279 bp, synthetic construct
  misc_feature 1..279: note = TAFA2_Varanus komodoensis
  source 1..279: mol_type = other DNA
gttaaaacggggacctgtgaagtggtggctctccaccggtgttgtaataagaacaagatagaagaaagatcacagacagtgaagtgctcctgctttcctgggcaggtagcaggtaccactcgagcagctccttcttgcgttgatgcttcaattgtggaacaaaaatggtggtgccacatgcagccatgtcttgaaggggaggaatgcaaagttcttccagatcgaaaaggatggagttgttcttctgggaataaagtgaaaacaacaagagtgagcaaa

SEQ ID NO: 209 - DNA, 273 bp, synthetic construct
  misc_feature 1..273: note = TAFA2_Podarcis muralis_isoform1
  source 1..273: mol_type = other DNA
gttaaaactggaacttgtgaagtggtggctctccaccgatgttgtaataagaacaagatagaagaaagatcgcagaccgtcaagtgctcctgcttccccgggcaggtagcaggtaccacacgagcagctccttcttgcgttgatgcttcaatagtggaacaaaaatggtggtgccacatgcagccatgtcttgaaggggaagaatgcaaagttcttccagatcggaaaggatggagttgttcttccggcaataaagtgaaaacaacaaggatg

SEQ ID NO: 210 - DNA, 279 bp, synthetic construct
  misc_feature 1..279: note = TAFA2_Podarcis muralis_isoform2
  source 1..279: mol_type = other DNA
gttaaaactggaacttgtgaagtggtggctctccaccgatgttgtaataagaacaagatagaagaaagatcgcagaccgtcaagtgctcctgcttccccgggcaggtagcaggtaccacacgagcagctccttcttgcgttgatgcttcaatagtggaacaaaaatggtggtgccacatgcagccatgtcttgaaggggaagaatgcaaagttcttccagatcggaaaggatggagttgttcttccggcaataaagtgaaaacaacaagggtaactcga

SEQ ID NO: 211 - DNA, 279 bp, synthetic construct
  misc_feature 1..279: note = TAFA2_Sceloporus undulatus
  source 1..279: mol_type = other DNA
gttaaaactggaacttgtgaagtggtggctctccatcggtgttgcaataagaacaagatagaagaaagatcacagacagtcaagtgctcctgctttcctgggcaggtagcaggtaccactcgagcagcgccttcttgtgttgatgcttcaatagtggaacaaaaatggtggtgccacatgcaaccatgtcttgaaggggaggaatgcaaagttcttccagatcgcaaaggatggagttgttcttctgggaataaagtgaaaacaacaagggtaactcga

SEQ ID NO: 212 - DNA, 276 bp, synthetic construct
  misc_feature 1..276: note = TAFA2_Gekko japonicus
  source 1..276: mol_type = other DNA
gttaaaactggaacttgtgaagtggtggctctccaccgatgttgtaataagaacaagatagaagaaagatcacagacagtcaaatgctcctgctttcctgggcaggtagctggtaccactcgagcagctccttcctgtgttgatgcttctatagtagaacaaaaatggtggtgtcaaatgcaaccatgccttgaaggtgaagagtgcaaagtccttccagataggaaaggatggagttgttcttctggaaataaggtgaaaacaacacgggcaaac

SEQ ID NO: 213 - DNA, 279 bp, synthetic construct
  misc_feature 1..279: note = TAFA2_Xenopus tropicalis
  source 1..279: mol_type = other DNA
gttagaactggaacttgtgaagttgtggccctacacagatgttgcaataaaaataagatagaagaaagatcccaaacagtcaagtgctcatgttttccaggacaagtggcagggacaacaagagcaactccttcttgtgtggatgcgtcaattgtcgagcagaaatggtggtgccatatgcagccgtgtcttgaaggtgaagaatgcaaaattcttccagatcagaaaggctggagttgtgcctcagggaataaagtgaaaacaacaaaggtaacacgg

SEQ ID NO: 214 - DNA, 279 bp, synthetic construct
  misc_feature 1..279: note = TAFA2_Danio rerio
  source 1..279: mol_type = other DNA
gtcaaagcgggaacctgtgaggtcattgctgcccaccgctgctgtaacaagaacaaaatcgaggagcgctcccaaactgtcaagtgctcctgcttccctgggcaagtggctggaacaacaagagctgctccatcctgtgtggacgcatctatagtagcgcagaagtggtggtgtcagatgcagccgtgtatggacggtgaggagtgtaaggtgttgccggatctaaaaggctggagctgcagcacaggcaacaaagtcaagacgaccaaggtcacacga

SEQ ID NO: 215 - DNA, 279 bp, synthetic construct
  misc_feature 1..279: note = TAFA3_Homo sapiens_isoform1
  source 1..279: mol_type = other DNA
gtgcagcagggcacctgcgaggtgattgcggctcaccgctgctgcaaccggaaccgcatcgaggagcgctcccagacggtgaaatgctcctgtttttctggccaggtggccggcaccacgcgggcaaagccctcctgcgtggacgcctccatcgtcctgcagagatggtggtgtcagatggagccctgcctgccgggggaggagtgtaaggtgctcccggacctgtcgggatggagctgcagcagtggacacaaagtcaaaaccaccaaggtcacacga

SEQ ID NO: 216 - DNA, 279 bp, synthetic construct
  misc_feature 1..279: note = TAFA3_Macaca fascicularis_isoform3
  source 1..279: mol_type = other DNA
gtgcagcagggcacctgcgaggtgattgcggctcaccgctgctgcaaccgaaaccgcatcgaggagcgctcccagacggtgaaatgctcctgtttttctggccaggtggccggcaccacgcgggcaaagccctcctgcgtggacgcctccatcgtcctgcagagatggtggtgtcagatggagccctgcctgccgggggaggagtgtaaggtgctcccggacctgtcgggatggagctgcagcagtggacacaaagtcaaaaccaccaaggtcacacga

SEQ ID NO: 217 - DNA, 279 bp, synthetic construct
  misc_feature 1..279: note = TAFA3_Sus scrofa_isoform2
  source 1..279: mol_type = other DNA
gtgaagcagggcacctgtgaggtgattgccgctcaccgctgctgtaaccggaaccgcatcgaggagcgctcccagactgtcaaatgctcttgcttttctggccaggtggccggcaccacccgggcaaagccctcctgcgtggatgcctccatcgtcctgcagaagtggtggtgccagatggagccctgcctgcctggggaggagtgtaaagtgctcccggacctgtcaggatggagctgcagcagtggacacaaagtcaaaaccaccaaggttacaaga

SEQ ID NO: 218 - DNA, 279 bp, synthetic construct
  misc_feature 1..279: note = TAFA3_Oryctolagus cuniculus_isoform2
  source 1..279: mol_type = other DNA
gtgaagcagggaacctgcgaggtgatcgccgctcatcgctgctgcaaccagaaccgcattgaggagcgctcccagaccgtcaaatgctcctgcctttcgggccaggtggccggcaccacccgggccaagccctcctgcgtggacgcctccatcgtcctgcagaggtggtggtgtcagatggagccctgcctgccgggagaggagtgtaaggtgctcccggacctgtcggggtggagctgcagcagtggacacaaagtgaaaaccaccaaggtcacccga

SEQ ID NO: 219 - DNA, 279 bp, synthetic construct
  misc_feature 1..279: note = TAFA3_Rattus norvegicus
  source 1..279: mol_type = other DNA
gtgaagcagggcacctgtgaggtgattgccgcacatcgctgctgtaaccgcaaccgtatcgaggagcgctcccaaacggtcaaatgctcctgcctttctggccaggtggctggcacaacaagagcaaagccctcctgtgtggacgcgtccatcgtcctgcagaagtggtggtgtcagatggagccctgcttgctgggggaggagtgtaaggtgctcccggacctgtcagggtggagctgcagccgaggacacaaggtcaaaaccaccaaggtcacacgg

SEQ ID NO: 220 - DNA, 279 bp, synthetic construct
  misc_feature 1..279: note = TAFA3_Mus musculus_isoform1
  source 1..279: mol_type = other DNA
gtgaagcagggcacctgcgaggtgattgctgcacatcgctgctgcaaccggaaccgcattgaggagcgctcccagacggtcaaatgctcctgcctgtccggccaggtggctggcaccaccagagcaaagccctcctgcgtggacgcctccatcgtcctgcagaagtggtggtgtcagatggagccctgcctgctgggagaggagtgtaaggtgctcccggacctgtcagggtggagctgcagcagtggacacaaggtcaaaaccaccaaggtcacacgg

SEQ ID NO: 221 - DNA, 279 bp, synthetic construct
  misc_feature 1..279: note = TAFA3_Gallus gallus
  source 1..279: mol_type = other DNA
gtggagcccggcacctgcgaggtcatcgcagcacacaggtgctgcaataagaacaagatagaggagcgttcccagaccgtgaagtgctcctgcttccctgggcaggtggcgggcaccacgcgggcagccccctcctgtgtggatgcctccatcgtgctgcagaagtggtggtgccagatggagccctgcctcgccggggaggagtgcaaagtgctgcccgacctctcaggctggagttgcagcagcggcaacaaagtgaagaccaccaaggtcacccgg

SEQ ID NO: 222 - DNA, 279 bp, synthetic construct
  misc_feature 1..279: note = TAFA3_Varanus komodoensis_isoform2
  source 1..279: mol_type = other DNA
atagagcctggcacatgtgaagtcattgctgcccacagatgctgcaataagaacaagatcgaagagcgctcgcaaacagtgaaatgttcctgctttccaggtcaggtggctgggactacacgggctgctccttcatgtgtagatgcttcaattgtgcttcagaagtggtggtgccaaatgcagccatgtctagaaggcgaagaatgtaaggtgctaccagatttgtctggatggagctgcagtactggaaacaaagtgaagacaaccaaggttacaagg

SEQ ID NO: 223 - DNA, 279 bp, synthetic construct
  misc_feature 1..279: note = TAFA3_Podarcis muralis
  source 1..279: mol_type = other DNA
atagagcctggcacatgtgaagtcatcgctgctcacaggtgctgcaataagaacaagattgaggagcgctcacaaacagtgaaatgttcctgctttccaggtcaggtggctgggacgacgcacgctgctccttcatgtgtagacgcctcaatagtgcttcagaagtggtggtgccaaatgcaaccatgtgtagaaggagaagagtgtaaagtgctaccagatttgtccggatggagctgcagtactggaaacaaagtaaagaccaccaaggtgacaagg

SEQ ID NO: 224 - DNA, 279 bp, synthetic construct
  misc_feature 1..279: note = TAFA3_Sceloporus undulatus
  source 1..279: mol_type = other DNA
atagagcctggcacatgtgaagtcattgctgcccacagatgctgcaataagaacaagattgaagaacggtcacagacagtgaaatgttcctgttttccaggtcaggtggctgggaccacacgtgctgctccttcatgtgtagatgcttcaatagtgcttcagaagtggtggtgccaaatgcaaccatgtttagaaggagaagaatgtaaggtgctaccagatttatctggatggagctgcagtactggaaacaaagtaaagacaaccaaggtcacccgg

SEQ ID NO: 225 - DNA, 279 bp, synthetic construct
  misc_feature 1..279: note = TAFA3_Xenopus tropicalis_isoform2
  source 1..279: mol_type = other DNA
gttgaaccgggtacatgtgaagtaatcgctgcccatagatgctgcaataagaacaagattgaggagcggtcacaaacagtaaaatgctcttgttttcctggacaagttgcaggaaccacaagagcagcaccatcatgtgtcgatgcttctatagttatccagaagtggtggtgtcaaatggagccatgtttagaaggagaagactgcaaagttttaccagacttgtctggatggagttgtagtactggaaacaaagtaaaaacaacaaaggtcacccga

SEQ ID NO: 226 - DNA, 279 bp, synthetic construct
  misc_feature 1..279: note = TAFA3_Danio rerio
  source 1..279: mol_type = other DNA
gtgaaagctggcacatgtgaggtgattgcagcccatcgctgctgtaacagaaataagattgaggagcgatcgcagacggtcaagtgttcctgcttccccggacaagtggctggaacgacgagagctgcaccctcctgtgtggacgcatctatagtagctcagaagtggtggtgtcaaatgcagccatgtgtggatggtgaggagtgtaaagtcctgcccgacctcacaggctggagctgcagcacgggcaacaaggtgaagacaaccaaggtgactcga

SEQ ID NO: 227 - DNA, 279 bp, synthetic construct
  misc_feature 1..279: note = TAFA4_Macaca fascicularis_isoform2
  source 1..279: mol_type = other DNA
atcaagcagggtacctgtgaggtggtcgccgtgcacaggtgctgcaataagaaccgcatagaagagcggtcacaaacggtcaagtgctcttgcttcccgggacaggtggccggcacaactcgggctcaaccttcttgcgttgaagcttccattgtgattcagaaatggtggtgtcacatgaatccatgtttggaaggagaggattgtaaagtgctgccagattactcaggttggtcctgtagcagtggcaataaagtcaaaactacaaaggtaacgcgg

SEQ ID NO: 228 - DNA, 279 bp, synthetic construct
  misc_feature 1..279: note = TAFA4_Sus scrofa_isoform2
  source 1..279: mol_type = other DNA
atcaagcaagggacctgtgaggtggtcgcagtgcacaggtgctgtaacaagaaccgcattgaggagcgatcacaaacggtcaagtgttcttgcttcccaggacaggttgctggcacaactcgggctcagccttcttgtgttgaagcttccattgtgattcagaaatggtggtgtcacatgaatccttgtttggaaggagaggattgtaaagtgctgccagattactcaggttggtcctgtagcagtggcaataaagtcaaaactacaaaggtaacacgg

SEQ ID NO: 229 - DNA, 279 bp, synthetic construct
  misc_feature 1..279: note = TAFA4_Oryctolagus cuniculus_isoform4
  source 1..279: mol_type = other DNA
atcaagccagggacctgcgaggtggttgccgtgcaccgatgctgcaataagaaccgcatagaagagcggtcacagacggtcaagtgctcctgcttccctggacaggtggctggcacgactcaggcccagccttcgtgtgttgaagcttccatcgtggctcagaaatggtggtgtcacatgaatccttgtttggaaggagaggactgcaaagtactgccagattactcaggttggtcctgtagcagtggcaataaagtcaaaactacaaaggtcacacgg

SEQ ID NO: 230 - DNA, 279 bp, synthetic construct
  misc_feature 1..279: note = TAFA4_Rattus norvegicus
  source 1..279: mol_type = other DNA
atcaagcaaggtacgtgtgaggtggtcgctgtgcaccgctgctgcaataagaaccgcatagaggagcgctctcagacggtcaagtgttcctgcttcccaggtcaggtggctggcacaactcgggcacagccttcttgtgttgaagcttccattgtgattgagaagtggtggtgccacatggatccttgcttggaaggagaggactgtaaagtgcttccggactcctctggttggtcctgtagcagtggcaataaagtcaaaaccacaaaggtgacccgg

SEQ ID NO: 231 - DNA, 279 bp, synthetic construct
  misc_feature 1..279: note = TAFA4_Mus musculus
  source 1..279: mol_type = other DNA
atcaagccaggtacctgcgaggtggtcgccgtgcaccgctgctgcaataagaaccgcatagaggagcgctctcagacggtcaaatgttcctgcttcccaggccaggtggctggcacaactcgggcacagccttcttgtgttgaagctgccattgtgattgagaagtggtggtgccacatgaatccttgcttggaaggagaggactgtaaagtgcttccagactcttcgggttggtcctgtagcagtggcaataaagtcaaaaccaccaaggtgacccgg

SEQ ID NO: 232 - DNA, 279 bp, synthetic construct
  misc_feature 1..279: note = TAFA4_Gallus gallus
  source 1..279: mol_type = other DNA
gtcaagcaagggacatgcgaggttgtggcagtgcatcgttgctgcaataagaaccggattgaggagcgatcgcaaacagtcaagtgctcctgcttcccagggcaggtggctgggacaacgcgggctcagccctcgtgcgtggaagcttctattgtcctgcagaagtggtggtgtcatatgaacccctgtttggatggagaggactgtaaggtactaccagactactcagggtggtcttgcagcagtggaaataaagtcaaaaccacaaaggtaacgcgg

SEQ ID NO: 233 - DNA, 279 bp, synthetic construct
  misc_feature 1..279: note = TAFA4_Varanus komodoensis_isoform2
  source 1..279: mol_type = other DNA
gtgaagcaagggacgtgcgaagtggttgctgtgcaccggtgttgcaacaagaaccggatcgaagagcggtcgcaaacggtcaagtgctcttgcctcccggggcaggttgctggcacaacgagggcgcagccctcctgcgtcgaagctgctattgttgtccagaagtggtggtgtcatatgaacccttgtctggaaggagaagaatgtaaagtactgccagattattcaggttggtcgtgcagcagtggaaacaaagtcaaaactaccaaggtgacacgg

SEQ ID NO: 234 - DNA, 279 bp, synthetic construct
  misc_feature 1..279: note = TAFA4_Podarcis muralis
  source 1..279: mol_type = other DNA
gttaagcaagggacctgcgaagtggtggcagtgcatcggtgctgcaacaagaacaggattgaagagcggtcgcagacggtcaagtgctcctgcttcccgggtcaggtggctggcacaacaagagcgcagccctcctgcgtcgaagctgccattgtcatccagaagtggtggtgtcatatgaacccttgcctggacggagaagactgtaaagtgcttccagattactcaggttggtcatgcagcagtggaaacaaagtcaaaactaccaaggtaacacgg

SEQ ID NO: 235 - DNA, 279 bp, synthetic construct
  misc_feature 1..279: note = TAFA4_Sceloporus undulatus
  source 1..279: mol_type = other DNA
gtgaagcaaggaacatgcgaagtggttgcggtgcaccggtgttgcaacaagaacaggattgaagaacggtcacaaacagtcaagtgttcttgcttcccagggcaggttgctggcacaacgagatcccagccctcctgcgttgaagctgccattgtcattcagaagtggtggtgtcatatgaacccttgtctggaaggagaagaatgtaaagtacttccagattactcaggttggtcctgcagcagtggaaacaaagtcaaaactaccaaggtgacacgg

SEQ ID NO: 236 - DNA, 279 bp, synthetic construct
  misc_feature 1..279: note = TAFA4_Gekko japonicus
  source 1..279: mol_type = other DNA
gttaagcaagggacctgtgaagtggttgcagtgcatctgtgttgcaacaagaacaggattgaagagctgtctcagacaggcaactgttcttgcctcccagggcaagttgcgggtacaacacgaactcagccctcctgtgtggaagccgccattgtcatccagaagtggtggtgtcagatgagcccttgtctggaaggagaggaatgtaaagtgcttcctgattcctcagggtggtcctgcagcagtgggaataaagtcaaaactaccaaggtgacccgg

SEQ ID NO: 237 - DNA, 279 bp, synthetic construct
  misc_feature 1..279: note = TAFA4_Xenopus tropicalis
  source 1..279: mol_type = other DNA
gtaaagcaaggtacctgtgaggttgtcgcacttcatcgatgctgcaataagaaccgaattgaagaacgatcacaaaccgtgaagtgttcttgcttcccggggcaggttgccggcaccaccagggcccagccatcttgcgtggaggcttctatcgtgatccagaagtggtggtgtcacatgaatccctgtatggaaggggaagagtgcaaagtgttgcctgatctcacaggctggtcctgcagcagcggaaacaaaataaaaacgaccaaggtaacacgg

SEQ ID NO: 238 - DNA, 279 bp, synthetic construct
  misc_feature 1..279: note = TAFA4_Danio rerio
  source 1..279: mol_type = other DNA
gtaaagcagggtacctgtgaggtggttgccatccaccgctgctgcaataagaacaagattgaggagcgttcacagaccgtcaagtgctcatgtttccctggtcaggtggccggtaccacacgtgcacagccatcttgtgtggaggcttccatcgtgctacagaagtggtggtgccaaatgcacccatgtttggatggcgaggagtgcaaagctcttccagatctgactggctggtcctgcagcaccggtaacaaagtcaaaaccactaaggtcacacga

SEQ ID NO: 239 - DNA, 294 bp, synthetic construct
  misc_feature 1..294: note = TAFA1_Homo sapiens
  source 1..294: mol_type = other DNA
ctgcacagaccagaaggagggacgtgtgaagtgatagcagcacaccgatgttgtaacaagaatcgcattgaggagcggtcacaaacagtaaagtgttcctgtctacctggaaaagtggctggaacaacaagaaaccggccttcttgcgtcgatgcctccatagtgattgggaaatggtggtgtgagatggagccttgcctagaaggagaagaatgtaagacactccctgacaattctggatggatgtgcgcaacaggcaacaaaattaagaccacgagaattcacccaagaacc

SEQ ID NO: 240 - DNA, 294 bp, synthetic construct
  misc_feature 1..294: note = TAFA1_Macaca fascicularis_isoform1
  source 1..294: mol_type = other DNA
ctgcacagaccagaaggagggacgtgtgaagtgatagcagcacaccgatgttgtaacaagaatcgcattgaggagaggtcacaaacagtaaagtgttcctgtctacctggaaaagtggctggaacaacaagaaaccggccttcctgtgttgacgcctccatagtgattgggaaatggtggtgtgagatggagccttgcctagaaggagaagaatgtaagacactccctgacaattctggatggatgtgcgcaacaggcaacaaaattaagaccacgagaattcacccaagaacc

SEQ ID NO: 241 - DNA, 294 bp, synthetic construct
  misc_feature 1..294: note = TAFA1_Sus scrofa_isoform2
  source 1..294: mol_type = other DNA
ctgcacagaccagaaggagggacatgtgaagtgattgccgcacacagatgttgtaataagaatcgcattgaggagcggtcacaaacagtcaagtgttcctgtctacctgggaaagtggctggaacaacaagaaaccgaccttcctgtgttgatgcctccatagtgattgggaaatggtggtgtgagatggagccttgtctagaaggagaagaatgcaaaacactccctgataattctggatggatgtgtgctacaggcaataaaattaagaccacaagaattcacccaagaacc

SEQ ID NO: 242 - DNA, 294 bp, synthetic construct
  misc_feature 1..294: note = TAFA1_Oryctolagus cuniculus_isoform1
  source 1..294: mol_type = other DNA
ctgcacagaccagaaggagggacatgcgaggtgatagcagcacacagatgttgtaacaagaaccgcattgaggagcggtcgcaaacggtgaagtgttcctgtctccctgggaaagtggcaggaaccacaagaaaccgaccttcctgtgtggatgcctccattgtgattgggaaatggtggtgtgagatggagccttgtctagagggagaagaatgtaagacactccctgacaattctggatggatgtgcgcgacaggcaacaaaattaagaccacacgaatccatccaagaacc

SEQ ID NO: 243 - DNA, 294 bp, synthetic construct
  misc_feature 1..294: note = TAFA1_Rattus norvegicus_isoform1
  source 1..294: mol_type = other DNA
ctgcacaggccagaaggagggacctgtgaagtgatagcggcccacaggtgttgcaacaagaaccgcattgaggagcggtcacaaacagtgaagtgttcctgtctacctgggaaagtggctgggacaacaagaaaccgaccttcctgtgttgatgcctccatagtgattgggaaatggtggtgtgagatggaaccctgcctagaaggagaagaatgtaagacactccctgacaactctggatggatgtgtgctacaggcaacaagatcaagaccacacgaattcacccaagaacc

SEQ ID NO: 244 - DNA, 294 bp, synthetic construct
  misc_feature 1..294: note = TAFA1_Mus musculus
  source 1..294: mol_type = other DNA
ctgcaccggccagaaggagggacctgtgaagtgatcgcggcccacaggtgttgtaacaagaaccgcatcgaggagcggtcacaaacagtgaagtgttcctgtttacctgggaaagtggctgggacaacaagaaaccgaccttcctgtgtggatgcctccatagtaattgggaaatggtggtgtgagatggagccctgcctagaaggagaagaatgtaagacactccctgacaattctggatggatgtgtgctacaggcaacaagattaagactacacgaattcacccaagaacc

SEQ ID NO: 245 - DNA, 294 bp, synthetic construct
  misc_feature 1..294: note = TAFA1_Gallus gallus_isoform2
  source 1..294: mol_type = other DNA
ctgcacagaccagaaggaggaacgtgtgaagttatagcagcacacagatgctgtaataagaatcgaattgaggaaagatcacaaacagtaaaatgctcctgtctacctgggaaagtggctgggactacacgaaacagaccttcctgtgttgatgcttcaatagtgattgggaaatggtggtgtgagatggagccctgcctagaaggagaggaatgtaagacgttgcctgataattctggatggatgtgtgcgactggcaataaaatcaagaccaccagaatccacccaaggacc

SEQ ID NO: 246 - DNA, 294 bp, synthetic construct
  misc_feature 1..294: note = TAFA1_Varanus komodoensis
  source 1..294: mol_type = other DNA
ctgcacagaccagaagggggaacgtgtgaagttatagctgcacacagatgctgcaacaagaatcggattgaggagagatcacaaacagtaaagtgctcctgtctacctgggaaagtggctgggacaacgcggaacagaccatcatgtgttgacgcatcaatagtcattgggaaatggtggtgtgaaatggagccctgcctagagggtgaggaatgcaagacattgccggacaattcaggatggatgtgcgcaaccggcaataaagtcaagaccaccagaattcacccgagaacc

SEQ ID NO: 247 - DNA, 294 bp, synthetic construct
  misc_feature 1..294: note = TAFA1_Podarcis muralis_isoform1
  source 1..294: mol_type = other DNA
ctgcacagaccagaaggagggacgtgtgaagttatagcagcacacagatgttgtaataagaatcggattgaagagagatcacaaacagtaaaatgctcctgtctacctgggaaagtggccgggacgacgcggaacagaccgtcgtgtgttgatgcatcaatagtcattgggaaatggtggtgtgagatggagccatgcctagagggcgaggaatgcaagacgttacctgacaactcaggatggatgtgtgcaaccggcaataaagtcaagaccaccagaattcatccgagaacc

SEQ ID NO: 248 - DNA, 294 bp, synthetic construct
  misc_feature 1..294: note = TAFA1_Sceloporus undulatus_isoform1
  source 1..294: mol_type = other DNA
ctgcacagaccagaaggaggcacgtgtgaagttatagcagcacatagatgttgtaataagaatcggattgaggagagatcacaaacagtaaagtgctcctgtctacctggaaaagtggctggcacgacgcggaacagaccatcatgtgttgacgcgtccatagttattgggaaatggtggtgtgaaatggagccctgcctagagggtgaagaatgcaaaacattacctgacaattcaggatggatgtgtgcaactggcaataaagtcaagaccaccagaattcacccgcgaacc

SEQ ID NO: 249 - DNA, 342 bp, synthetic construct
  misc_feature 1..342: note = TAFA1_Xenopus tropicalis_isoform1
  source 1..342: mol_type = other DNA
ttgcaccaatcaggatttacttcaggacacttcccccatcacaggaaactgggagaaatagaaggtggaacctgtgaagttatagctgcgcacagatgctgcaataagaatcgcatcgaggaacgctcacagaccgtgaaatgttcttgtcttcctggaaaagtggctggaacgacacggaacaggccctcttgtgtcgatgcttccatagttattggaaaatggtggtgtgagatggaaccttgtttagaaggggaagaatgtaagacccttcccgacaactcgggctggatgtgtgccaccggcaataagatcaagaccacaagatttcagggtcactta

SEQ ID NO: 250 - DNA, 342 bp, synthetic construct
  misc_feature 1..342: note = TAFA1_Xenopus tropicalis_isoform2
  source 1..342: mol_type = other DNA
ttgcaccaatcaggatttacttcaggacacttcccccatcacaggaaactgggagaaatagaaggtggaacctgtgaagttatagctgcgcacagatgctgcaataagaatcgcatcgaggaacgctcacagaccgtgaaatgttcttgtcttcctggaaaagtggctggaacgacacggaacaggccctcttgtgtcgatgcttccatagttattggaaaatggtggtgtgagatggaaccttgtttagaaggggaagaatgtaagacccttcccgacaactcgggctggatgtgtgccaccggcaataagatcaagaccacaagaattcacccgagatcc

SEQ ID NO: 251 - DNA, 327 bp, synthetic construct
  misc_feature 1..327: note = TAFA1_Danio rerio_isoform1
  source 1..327: mol_type = other DNA
ctggcaccgcctggaaccaacatacagatcctcgaaggagggacatgcgaggtgatcgcggcgcacaggtgctgtaacaaaaacaagattgaagagagatctcagacagtgaagtgctcctgtttacctgggaaagtggcaggaaccaccaggaacaaaccctcctgtgttgacgcctccattgtgattgggaagtggtggtgtgagatggagccgtgtctggagggagaagagtgtaagactctaccagacaactccggctggatgtgctactctggaaacaagatcaaaaccaccaggggaaacatccaagaggacaagctgaaa

SEQ ID NO: 252 - DNA, 324 bp, synthetic construct
  misc_feature 1..324: note = TAFA1_Danio rerio_isoform2
  source 1..324: mol_type = other DNA
ctggcaccgcctggaaccaacatacagatcctcgaaggagggacatgcgaggtgatcgcggcgcacaggtgctgtaacaaaaacaagattgaagagagatctcagacagtgaagtgctcctgtttacctgggaaagtggcaggaaccaccaggaacaaaccctcctgtgttgacgcctccattgtgattgggaagtggtggtgtgagatggagccgtgtctggagggagaagagtgtaagactctaccagacaactccggctggatgtgctactctggaaacaagatcaaaaccaccaggaatacccacccatacacatccttg

SEQ ID NO: 253 - DNA, 303 bp, synthetic construct
  misc_feature 1..303: note = TAFA2_Homo sapiens
  source 1..303: mol_type = other DNA
gcaaaccatcataaagctcaccatgttaaaacgggaacttgtgaggtggtggcactccacagatgctgtaataagaacaagatagaagaacggtcacaaacagtcaagtgctcctgcttccctgggcaggtggcaggcaccacgcgagctgctccatcatgtgtggatgcttcaatagtggaacagaaatggtggtgccatatgcagccatgtctagagggagaagaatgtaaagttcttccggatcggaaaggatggagctgttcctctgggaataaagtcaaaacaactagggtaacccat

SEQ ID NO: 254 - DNA, 303 bp, synthetic construct
  misc_feature 1..303: note = TAFA2_Macaca fascicularis
  source 1..303: mol_type = other DNA
gcaaaccatcataaagctcaccatgttaaaacgggaacttgtgaggtggtggcactccacagatgctgtaataagaacaagatagaagaacggtcacaaacagtcaagtgctcctgcttccccgggcaggtggcaggcaccacgcgagctgctccatcatgtgtggatgcttcaatagtggaacagaaatggtggtgccatatgcagccatgtctagagggagaagaatgtaaagttcttccagatcggaaaggatggagctgttcctctgggaataaagtcaaaacaactagggtaacccat

SEQ ID NO: 255 - DNA, 303 bp, synthetic construct
  misc_feature 1..303: note = TAFA2_Sus scrofa
  source 1..303: mol_type = other DNA
gtaaaccatcataaagctcaccatgttaaaacgggcacttgtgaggtggtggcactccacagatgctgtaataagaacaagatagaagaacggtcacaaacagtcaagtgctcctgcttccctgggcaggtggcaggcaccacacgggctgctccatcttgtgtggatgcttcaatagtggaacagaaatggtggtgccatatgcaaccgtgtcttgagggagaggaatgtaaagttcttccagatcggaaaggatggagctgttcctctgggaataaagtgaaaacaacaagggtaacccat

SEQ ID NO: 256 - DNA, 303 bp, synthetic construct
  misc_feature 1..303: note = TAFA2_Oryctolagus cuniculus
  source 1..303: mol_type = other DNA
gcaaaccatcataaagctcatcatgttaaaacgggaacttgtgaggtggtggcactccacagatgctgtaataagaacaagatagaagaacggtcacaaactgtcaaatgctcctgcttcccggggcaggtggccggcaccacgcgagctgctccatcttgtgtggatgcttcaatagtagagcagaaatggtggtgccatatgcagccatgtctagagggagaagaatgtaaagttcttcctgatcggaaaggatggagctgttcctctgggaataaagtgaaaactactagagtaacccat

SEQ ID NO: 257 - DNA, 303 bp, synthetic construct
  misc_feature 1..303: note = TAFA2_Rattus norvegicus_isoform1
  source 1..303: mol_type = other DNA
gccaaccatcacaaagctcaccatgttagaactgggacttgcgaggtggtggcgctgcacagatgctgtaataagaacaagatagaagaacggtcccaaacggtcaagtgctcctgcttccctgggcaggtggcaggcactacccgagctgccccatcttgtgtggatgcatccatagtggaacaaaaatggtggtgtcatatgcagccatgtctggagggagaggaatgtaaagtccttccagatcgcaaaggatggagctgttcctctggaaacaaagtaaaaacaactagggcaaacgtg

SEQ ID NO: 258 - DNA, 303 bp, synthetic construct
  misc_feature 1..303: note = TAFA2_Rattus norvegicus_isoform2
  source 1..303: mol_type = other DNA
gccaaccatcacaaagctcaccatgttagaactgggacttgcgaggtggtggcgctgcacagatgctgtaataagaacaagatagaagaacggtcccaaacggtcaagtgctcctgcttccctgggcaggtggcaggcactacccgagctgccccatcttgtgtggatgcatccatagtggaacaaaaatggtggtgtcatatgcagccatgtctggagggagaggaatgtaaagtccttccagatcgcaaaggatggagctgttcctctggaaacaaagtaaaaacaactagggtaactcat

SEQ ID NO: 259 - DNA, 303 bp, synthetic construct
  misc_feature 1..303: note = TAFA2_Mus musculus_isoform1
  source 1..303: mol_type = other DNA
gccaaccatcacaaagctcaccatgttagaactgggacttgcgaggttgtggcgctgcacagatgctgtaataagaacaagatagaagaacggtcccaaacggtcaagtgctcctgcttccctgggcaggtggcaggcactacccgagctgctccgtcttgtgtggatgcatccatagtggaacaaaagtggtggtgtcatatgcagccatgcctggagggagaggaatgtaaagtccttccagatcgcaaaggatggagctgttcctctggaaacaaagtaaaaacaactagggtaacccat

SEQ ID NO: 260 - DNA, 303 bp, synthetic construct
  misc_feature 1..303: note = TAFA2_Gallus gallus_isoform1
  source 1..303: mol_type = other DNA
gcaaatcatcataaagctcaccatgttaaaactgggacctgtgaagtggtggcactccacagatgttgcaataagaacaagatagaagaaagatcacagacagtgaagtgctcctgcttccctgggcaggtagcaggtaccactcgggcagctccttcttgtgttgatgcttcaatagtggagcagaaatggtggtgccacatgcaaccatgtcttgaaggggaggaatgtaaggttcttccagatcgtaagggatggagctgttcctccgggaataaagtgaaaacaactagggcaaacgtg

SEQ ID NO: 261 - DNA, 303 bp, synthetic construct
  misc_feature 1..303: note = TAFA2_Gallus gallus_isoform2
  source 1..303: mol_type = other DNA
gcaaatcatcataaagctcaccatgttaaaactgggacctgtgaagtggtggcactccacagatgttgcaataagaacaagatagaagaaagatcacagacagtgaagtgctcctgcttccctgggcaggtagcaggtaccactcgggcagctccttcttgtgttgatgcttcaatagtggagcagaaatggtggtgccacatgcaaccatgtcttgaaggggaggaatgtaaggttcttccagatcgtaagggatggagctgttcctccgggaataaagtgaaaacaactagggtaacccga

SEQ ID NO: 262 - DNA, 357 bp, synthetic construct
  misc_feature 1..357: note = TAFA2_Varanus komodoensis
  source 1..357: mol_type = other DNA
gcaaaccatcacaaagctcatcatgttaaaacggggacctgtgaagtggtggctctccaccggtgttgtaataagaacaagatagaagaaagatcacagacagtgaagtgctcctgctttcctgggcaggtagcaggtaccactcgagcagctccttcttgcgttgatgcttcaattgtggaacaaaaatggtggtgccacatgcagccatgtcttgaaggggaggaatgcaaagttcttccagatcgaaaaggatggagttgttcttctgggaataaagtgaaaacaacaagagtgagcaaacgtgtaaaacccttcaagaacaaggagatttctgctgtgcctgatgacaatttt

SEQ ID NO: 263 - DNA, 318 bp, synthetic construct
  misc_feature 1..318: note = TAFA2_Podarcis muralis_isoform1
  source 1..318: mol_type = other DNA
gcaaaccaccacaaagctcaccatgttaaaactggaacttgtgaagtggtggctctccaccgatgttgtaataagaacaagatagaagaaagatcgcagaccgtcaagtgctcctgcttccccgggcaggtagcaggtaccacacgagcagctccttcttgcgttgatgcttcaatagtggaacaaaaatggtggtgccacatgcagccatgtcttgaaggggaagaatgcaaagttcttccagatcggaaaggatggagttgttcttccggcaataaagtgaaaacaacaaggatgttttggtgttgtgcgacagaa

SEQ ID NO: 264 - DNA, 303 bp, synthetic construct
  misc_feature 1..303: note = TAFA2_Podarcis muralis_isoform2
  source 1..303: mol_type = other DNA
gcaaaccaccacaaagctcaccatgttaaaactggaacttgtgaagtggtggctctccaccgatgttgtaataagaacaagatagaagaaagatcgcagaccgtcaagtgctcctgcttccccgggcaggtagcaggtaccacacgagcagctccttcttgcgttgatgcttcaatagtggaacaaaaatggtggtgccacatgcagccatgtcttgaaggggaagaatgcaaagttcttccagatcggaaaggatggagttgttcttccggcaataaagtgaaaacaacaagggtaactcga

SEQ ID NO: 265 - DNA, 303 bp, synthetic construct
  misc_feature 1..303: note = TAFA2_Sceloporus undulatus
  source 1..303: mol_type = other DNA
gcaaaccaccacaaagctcatcatgttaaaactggaacttgtgaagtggtggctctccatcggtgttgcaataagaacaagatagaagaaagatcacagacagtcaagtgctcctgctttcctgggcaggtagcaggtaccactcgagcagcgccttcttgtgttgatgcttcaatagtggaacaaaaatggtggtgccacatgcaaccatgtcttgaaggggaggaatgcaaagttcttccagatcgcaaaggatggagttgttcttctgggaataaagtgaaaacaacaagggtaactcga

SEQ ID NO: 266 - DNA, 303 bp, synthetic construct
  misc_feature 1..303: note = TAFA2_Gekko japonicus
  source 1..303: mol_type = other DNA
gcaaaccatcacaaagctcatcatgttaaaactggaacttgtgaagtggtggctctccaccgatgttgtaataagaacaagatagaagaaagatcacagacagtcaaatgctcctgctttcctgggcaggtagctggtaccactcgagcagctccttcctgtgttgatgcttctatagtagaacaaaaatggtggtgtcaaatgcaaccatgccttgaaggtgaagagtgcaaagtccttccagataggaaaggatggagttgttcttctggaaataaggtgaaaacaacacgggcaaacgtg

SEQ ID NO: 267 - DNA, 303 bp, synthetic construct
  misc_feature 1..303: note = TAFA2_Xenopus tropicalis
  source 1..303: mol_type = other DNA
gtaattcatcacaaagctcagcatgttagaactggaacttgtgaagttgtggccctacacagatgttgcaataaaaataagatagaagaaagatcccaaacagtcaagtgctcatgttttccaggacaagtggcagggacaacaagagcaactccttcttgtgtggatgcgtcaattgtcgagcagaaatggtggtgccatatgcagccgtgtcttgaaggtgaagaatgcaaaattcttccagatcagaaaggctggagttgtgcctcagggaataaagtgaaaacaacaaaggtaacacgg

SEQ ID NO: 268 - DNA, 309 bp, synthetic construct
  misc_feature 1..309: note = TAFA3_Homo sapiens_isoform1
  source 1..309: mol_type = other DNA
gccttgcagcctcccactgccacagtgcttgtgcagcagggcacctgcgaggtgattgcggctcaccgctgctgcaaccggaaccgcatcgaggagcgctcccagacggtgaaatgctcctgtttttctggccaggtggccggcaccacgcgggcaaagccctcctgcgtggacgcctccatcgtcctgcagagatggtggtgtcagatggagccctgcctgccgggggaggagtgtaaggtgctcccggacctgtcgggatggagctgcagcagtggacacaaagtcaaaaccaccaaggtcacacga

SEQ ID NO: 269 - DNA, 309 bp, synthetic construct
  misc_feature 1..309: note = TAFA3_Macaca fascicularis_isoform3
  source 1..309: mol_type = other DNA
gccttgcagcctcccactgctacagtgcttgtgcagcagggcacctgcgaggtgattgcggctcaccgctgctgcaaccgaaaccgcatcgaggagcgctcccagacggtgaaatgctcctgtttttctggccaggtggccggcaccacgcgggcaaagccctcctgcgtggacgcctccatcgtcctgcagagatggtggtgtcagatggagccctgcctgccgggggaggagtgtaaggtgctcccggacctgtcgggatggagctgcagcagtggacacaaagtcaaaaccaccaaggtcacacga

SEQ ID NO: 270 - DNA, 309 bp, synthetic construct
  misc_feature 1..309: note = TAFA3_Sus scrofa_isoform2
  source 1..309: mol_type = other DNA
tccttgcagcttccaactcccacagtccttgtgaagcagggcacctgtgaggtgattgccgctcaccgctgctgtaaccggaaccgcatcgaggagcgctcccagactgtcaaatgctcttgcttttctggccaggtggccggcaccacccgggcaaagccctcctgcgtggatgcctccatcgtcctgcagaagtggtggtgccagatggagccctgcctgcctggggaggagtgtaaagtgctcccggacctgtcaggatggagctgcagcagtggacacaaagtcaaaaccaccaaggttacaaga

SEQ ID NO: 271 - DNA, 309 bp, synthetic construct
  misc_feature 1..309: note = TAFA3_Oryctolagus cuniculus_isoform2
  source 1..309: mol_type = other DNA
tccttagagcctccaactactgcagtcctggtgaagcagggaacctgcgaggtgatcgccgctcatcgctgctgcaaccagaaccgcattgaggagcgctcccagaccgtcaaatgctcctgcctttcgggccaggtggccggcaccacccgggccaagccctcctgcgtggacgcctccatcgtcctgcagaggtggtggtgtcagatggagccctgcctgccgggagaggagtgtaaggtgctcccggacctgtcggggtggagctgcagcagtggacacaaagtgaaaaccaccaaggtcacccga

SEQ ID NO: 272 - DNA, 309 bp, synthetic construct
  misc_feature 1..309: note = TAFA3_Rattus norvegicus
  source 1..309: mol_type = other DNA
tccttgcagcctccaacatccacagtcctagtgaagcagggcacctgtgaggtgattgccgcacatcgctgctgtaaccgcaaccgtatcgaggagcgctcccaaacggtcaaatgctcctgcctttctggccaggtggctggcacaacaagagcaaagccctcctgtgtggacgcgtccatcgtcctgcagaagtggtggtgtcagatggagccctgcttgctgggggaggagtgtaaggtgctcccggacctgtcagggtggagctgcagccgaggacacaaggtcaaaaccaccaaggtcacacgg

SEQ ID NO: 273 - DNA, 309 bp, synthetic construct
  misc_feature 1..309: note = TAFA3_Mus musculus_isoform1
  source 1..309: mol_type = other DNA
tccttgcagcctccaacatccgcagtcctagtgaagcagggcacctgcgaggtgattgctgcacatcgctgctgcaaccggaaccgcattgaggagcgctcccagacggtcaaatgctcctgcctgtccggccaggtggctggcaccaccagagcaaagccctcctgcgtggacgcctccatcgtcctgcagaagtggtggtgtcagatggagccctgcctgctgggagaggagtgtaaggtgctcccggacctgtcagggtggagctgcagcagtggacacaaggtcaaaaccaccaaggtcacacgg

SEQ ID NO: 274 - DNA, 309 bp, synthetic construct
  misc_feature 1..309: note = TAFA3_Gallus gallus
  source 1..309: mol_type = other DNA
tccacccaccacagaagccattcagcacacgtggagcccggcacctgcgaggtcatcgcagcacacaggtgctgcaataagaacaagatagaggagcgttcccagaccgtgaagtgctcctgcttccctgggcaggtggcgggcaccacgcgggcagccccctcctgtgtggatgcctccatcgtgctgcagaagtggtggtgccagatggagccctgcctcgccggggaggagtgcaaagtgctgcccgacctctcaggctggagttgcagcagcggcaacaaagtgaagaccaccaaggtcacccgg

SEQ ID NO: 275 - DNA, 309 bp, synthetic construct
  misc_feature 1..309: note = TAFA3_Varanus komodoensis_isoform2
  source 1..309: mol_type = other DNA
tcatcacaccacagaagccattcagtgcacatagagcctggcacatgtgaagtcattgctgcccacagatgctgcaataagaacaagatcgaagagcgctcgcaaacagtgaaatgttcctgctttccaggtcaggtggctgggactacacgggctgctccttcatgtgtagatgcttcaattgtgcttcagaagtggtggtgccaaatgcagccatgtctagaaggcgaagaatgtaaggtgctaccagatttgtctggatggagctgcagtactggaaacaaagtgaagacaaccaaggttacaagg

SEQ ID NO: 276 - DNA, 309 bp, synthetic construct
  misc_feature 1..309: note = TAFA3_Podarcis muralis
  source 1..309: mol_type = other DNA
tcatcacaccacagaagccattcagtgcacatagagcctggcacatgtgaagtcatcgctgctcacaggtgctgcaataagaacaagattgaggagcgctcacaaacagtgaaatgttcctgctttccaggtcaggtggctgggacgacgcacgctgctccttcatgtgtagacgcctcaatagtgcttcagaagtggtggtgccaaatgcaaccatgtgtagaaggagaagagtgtaaagtgctaccagatttgtccggatggagctgcagtactggaaacaaagtaaagaccaccaaggtgacaagg

SEQ ID NO: 277 - DNA, 309 bp, synthetic construct
  misc_feature 1..309: note = TAFA3_Sceloporus undulatus
  source 1..309: mol_type = other DNA
tcatcacaccacagaagccattcagtgcacatagagcctggcacatgtgaagtcattgctgcccacagatgctgcaataagaacaagattgaagaacggtcacagacagtgaaatgttcctgttttccaggtcaggtggctgggaccacacgtgctgctccttcatgtgtagatgcttcaatagtgcttcagaagtggtggtgccaaatgcaaccatgtttagaaggagaagaatgtaaggtgctaccagatttatctggatggagctgcagtactggaaacaaagtaaagacaaccaaggtcacccgg

SEQ ID NO: 278 - DNA, 309 bp, synthetic construct
  misc_feature 1..309: note = TAFA3_Xenopus tropicalis_isoform2
  source 1..309: mol_type = other DNA
tcgtcacaccacagaattcattcagttcacgttgaaccgggtacatgtgaagtaatcgctgcccatagatgctgcaataagaacaagattgaggagcggtcacaaacagtaaaatgctcttgttttcctggacaagttgcaggaaccacaagagcagcaccatcatgtgtcgatgcttctatagttatccagaagtggtggtgtcaaatggagccatgtttagaaggagaagactgcaaagttttaccagacttgtctggatggagttgtagtactggaaacaaagtaaaaacaacaaaggtcacccga

SEQ ID NO: 279 - DNA, 306 bp, synthetic construct
  misc_feature 1..306: note = TAFA3_Danio rerio
  source 1..306: mol_type = other DNA
tcttctcaccgcagtcacatcgtgcacgtgaaagctggcacatgtgaggtgattgcagcccatcgctgctgtaacagaaataagattgaggagcgatcgcagacggtcaagtgttcctgcttccccggacaagtggctggaacgacgagagctgcaccctcctgtgtggacgcatctatagtagctcagaagtggtggtgtcaaatgcagccatgtgtggatggtgaggagtgtaaagtcctgcccgacctcacaggctggagctgcagcacgggcaacaaggtgaagacaaccaaggtgactcga

SEQ ID NO: 280 - DNA, 285 bp, synthetic construct
  misc_feature 1..285: note = TAFA4_Homo sapiens
  source 1..285: mol_type = other DNA
caccaaatcaagcaagggacctgtgaggtggtcgccgtgcacaggtgctgcaataagaaccgcatagaagagcggtcacaaacggtcaagtgctcttgcttcccgggacaggtggcgggcacaactcgggctcaaccttcttgtgttgaagcttccattgtgattcagaaatggtggtgtcacatgaatccgtgtttggaaggagaggattgtaaagtgctgccagattactcaggttggtcctgtagcagtggcaataaagtcaaaactacgaaggtaacgcgg

SEQ ID NO: 281 - DNA, 285 bp, synthetic construct
  misc_feature 1..285: note = TAFA4_Macaca fascicularis_isoform2
  source 1..285: mol_type = other DNA
caccaaatcaagcagggtacctgtgaggtggtcgccgtgcacaggtgctgcaataagaaccgcatagaagagcggtcacaaacggtcaagtgctcttgcttcccgggacaggtggccggcacaactcgggctcaaccttcttgcgttgaagcttccattgtgattcagaaatggtggtgtcacatgaatccatgtttggaaggagaggattgtaaagtgctgccagattactcaggttggtcctgtagcagtggcaataaagtcaaaactacaaaggtaacgcgg

SEQ ID NO: 282 - DNA, 285 bp, synthetic construct
  misc_feature 1..285: note = TAFA4_Sus scrofa_isoform2
  source 1..285: mol_type = other DNA
caccagatcaagcaagggacctgtgaggtggtcgcagtgcacaggtgctgtaacaagaaccgcattgaggagcgatcacaaacggtcaagtgttcttgcttcccaggacaggttgctggcacaactcgggctcagccttcttgtgttgaagcttccattgtgattcagaaatggtggtgtcacatgaatccttgtttggaaggagaggattgtaaagtgctgccagattactcaggttggtcctgtagcagtggcaataaagtcaaaactacaaaggtaacacgg

SEQ ID NO: 283 - DNA, 285 bp, synthetic construct
  misc_feature 1..285: note = TAFA4_Oryctolagus cuniculus_isoform4
  source 1..285: mol_type = other DNA
caccagatcaagccagggacctgcgaggtggttgccgtgcaccgatgctgcaataagaaccgcatagaagagcggtcacagacggtcaagtgctcctgcttccctggacaggtggctggcacgactcaggcccagccttcgtgtgttgaagcttccatcgtggctcagaaatggtggtgtcacatgaatccttgtttggaaggagaggactgcaaagtactgccagattactcaggttggtcctgtagcagtggcaataaagtcaaaactacaaaggtcacacgg

SEQ ID NO: 284 - DNA, 285 bp, synthetic construct
  misc_feature 1..285: note = TAFA4_Rattus norvegicus
  source 1..285: mol_type = other DNA
catgtgatcaagcaaggtacgtgtgaggtggtcgctgtgcaccgctgctgcaataagaaccgcatagaggagcgctctcagacggtcaagtgttcctgcttcccaggtcaggtggctggcacaactcgggcacagccttcttgtgttgaagcttccattgtgattgagaagtggtggtgccacatggatccttgcttggaaggagaggactgtaaagtgcttccggactcctctggttggtcctgtagcagtggcaataaagtcaaaaccacaaaggtgacccgg

SEQ ID NO: 285 - DNA, 285 bp, synthetic construct
  misc_feature 1..285: note = TAFA4_Mus musculus
  source 1..285: mol_type = other DNA
cacctgatcaagccaggtacctgcgaggtggtcgccgtgcaccgctgctgcaataagaaccgcatagaggagcgctctcagacggtcaaatgttcctgcttcccaggccaggtggctggcacaactcgggcacagccttcttgtgttgaagctgccattgtgattgagaagtggtggtgccacatgaatccttgcttggaaggagaggactgtaaagtgcttccagactcttcgggttggtcctgtagcagtggcaataaagtcaaaaccaccaaggtgacccgg

SEQ ID NO: 286 - DNA, 285 bp, synthetic construct
  misc_feature 1..285: note = TAFA4_Gallus gallus
  source 1..285: mol_type = other DNA
caccaagtcaagcaagggacatgcgaggttgtggcagtgcatcgttgctgcaataagaaccggattgaggagcgatcgcaaacagtcaagtgctcctgcttcccagggcaggtggctgggacaacgcgggctcagccctcgtgcgtggaagcttctattgtcctgcagaagtggtggtgtcatatgaacccctgtttggatggagaggactgtaaggtactaccagactactcagggtggtcttgcagcagtggaaataaagtcaaaaccacaaaggtaacgcgg

SEQ ID NO: 287 - DNA, 285 bp, synthetic construct
  misc_feature 1..285: note = TAFA4_Varanus komodoensis_isoform2
  source 1..285: mol_type = other DNA
caccaagtgaagcaagggacgtgcgaagtggttgctgtgcaccggtgttgcaacaagaaccggatcgaagagcggtcgcaaacggtcaagtgctcttgcctcccggggcaggttgctggcacaacgagggcgcagccctcctgcgtcgaagctgctattgttgtccagaagtggtggtgtcatatgaacccttgtctggaaggagaagaatgtaaagtactgccagattattcaggttggtcgtgcagcagtggaaacaaagtcaaaactaccaaggtgacacgg

SEQ ID NO: 288 - DNA, 285 bp, synthetic construct
  misc_feature 1..285: note = TAFA4_Podarcis muralis
  source 1..285: mol_type = other DNA
caccaagttaagcaagggacctgcgaagtggtggcagtgcatcggtgctgcaacaagaacaggattgaagagcggtcgcagacggtcaagtgctcctgcttcccgggtcaggtggctggcacaacaagagcgcagccctcctgcgtcgaagctgccattgtcatccagaagtggtggtgtcatatgaacccttgcctggacggagaagactgtaaagtgcttccagattactcaggttggtcatgcagcagtggaaacaaagtcaaaactaccaaggtaacacgg

SEQ ID NO: 289 - DNA, 285 bp, synthetic construct
  misc_feature 1..285: note = TAFA4_Sceloporus undulatus
  source 1..285: mol_type = other DNA
caccaagtgaagcaaggaacatgcgaagtggttgcggtgcaccggtgttgcaacaagaacaggattgaagaacggtcacaaacagtcaagtgttcttgcttcccagggcaggttgctggcacaacgagatcccagccctcctgcgttgaagctgccattgtcattcagaagtggtggtgtcatatgaacccttgtctggaaggagaagaatgtaaagtacttccagattactcaggttggtcctgcagcagtggaaacaaagtcaaaactaccaaggtgacacgg

SEQ ID NO: 290 - DNA, 285 bp, synthetic construct
  misc_feature 1..285: note = TAFA4_Gekko japonicus
  source 1..285: mol_type = other DNA
caccaagttaagcaagggacctgtgaagtggttgcagtgcatctgtgttgcaacaagaacaggattgaagagctgtctcagacaggcaactgttcttgcctcccagggcaagttgcgggtacaacacgaactcagccctcctgtgtggaagccgccattgtcatccagaagtggtggtgtcagatgagcccttgtctggaaggagaggaatgtaaagtgcttcctgattcctcagggtggtcctgcagcagtgggaataaagtcaaaactaccaaggtgacccgg

SEQ ID NO: 291 - DNA, 285 bp, synthetic construct
  misc_feature 1..285: note = TAFA4_Xenopus tropicalis
  source 1..285: mol_type = other DNA
tatcaagtaaagcaaggtacctgtgaggttgtcgcacttcatcgatgctgcaataagaaccgaattgaagaacgatcacaaaccgtgaagtgttcttgcttcccggggcaggttgccggcaccaccagggcccagccatcttgcgtggaggcttctatcgtgatccagaagtggtggtgtcacatgaatccctgtatggaaggggaagagtgcaaagtgttgcctgatctcacaggctggtcctgcagcagcggaaacaaaataaaaacgaccaaggtaacacgg

SEQ ID NO: 292 - DNA, 285 bp, synthetic construct
  misc_feature 1..285: note = TAFA4_Danio rerio
  source 1..285: mol_type = other DNA
taccaggtaaagcagggtacctgtgaggtggttgccatccaccgctgctgcaataagaacaagattgaggagcgttcacagaccgtcaagtgctcatgtttccctggtcaggtggccggtaccacacgtgcacagccatcttgtgtggaggcttccatcgtgctacagaagtggtggtgccaaatgcacccatgtttggatggcgaggagtgcaaagctcttccagatctgactggctggtcctgcagcaccggtaacaaagtcaaaaccactaaggtcacacga

SEQ ID NO: 293 - protein, 4 aa, synthetic construct
  REGION 1..4: note = TAFA1_LHRP
LHRP

SEQ ID NO: 294 - protein, 19 aa, synthetic construct
  REGION 1..19: note = TAFA1_LHQSGFTSGHFPHHRKLGE
LHQSGFTSGHFPHHRKLGE

SEQ ID NO: 295 - protein, 10 aa, synthetic construct
  REGION 1..10: note = TAFA1_LAPPGTNIQI
LAPPGTNIQI

SEQ ID NO: 296 - protein, 5 aa, synthetic construct
  REGION 1..5: note = TAFA1_PYTSL
PYTSL

SEQ ID NO: 297 - protein, 6 aa, synthetic construct
  REGION 1..6: note = TAFA1_QEDKLK
QEDKLK

SEQ ID NO: 298 - protein, 135 aa, synthetic construct
  REGION 1..135: note = TAFA4_Mus musculus
MRVCAKWVLLSRWLVLTYVLMVCCKLMSASSQHLRGHAGHHLIKPGTCEVVAVHRCCNKNRIEERSQTVKCSCFPGQVAGTTRAQPSCVEAAIVIEKWWCHMNPCLEGEDCKVLPDSSGWSCSSGNKVKTTKVTR

SEQ ID NO: 299 - protein, 140 aa, synthetic construct
  REGION 1..140: note = TAFA4_Homo sapiens
MRSPRMRVCAKSVLLSHWLFLAYVLMVCCKLMSASSQHLRGHAGHHQIKQGTCEVVAVHRCCNKNRIEERSQTVKCSCFPGQVAGTTRAQPSCVEASIVIQKWWCHMNPCLEGEDCKVLPDYSGWSCSSGNKVKTTKVTR

SEQ ID NO: 300 - protein, 135 aa, synthetic construct
  REGION 1..135: note = TAFA4_Gekko japonicus
MRFCAKSMLPSQWLFLAYVLMVCCKSLSATSYHPRGHPGHHQVKQGTCEVVAVHLCCNKNRIEELSQTGNCSCLPGQVAGTTRTQPSCVEAAIVIQKWWCQMSPCLEGEECKVLPDSSGWSCSSGNKVKTTKVTR

SEQ ID NO: 301 - protein, 135 aa, synthetic construct
  REGION 1..135: note = TAFA4_Danio rerio
MQLWGRSLWPLRIVLLFTLVMCSCGLVSAGTRSLRGHTASYQVKQGTCEVVAIHRCCNKNKIEERSQTVKCSCFPGQVAGTTRAQPSCVEASIVLQKWWCQMHPCLDGEECKALPDLTGWSCSTGNKVKTTKVTR

SEQ ID NO: 302 - protein, 133 aa, synthetic construct [sequence omitted]

SEQ ID NO: 303 - protein, 131 aa, synthetic construct
  REGION 1..131: note = TAFA2_Homo sapiens
MSKRYLQKATKGKLLIIIFIVTLWGKVVSSANHHKAHHVKTGTCEVVALHRCCNKNKIEERSQTVKCSCFPGQVAGTTRAAPSCVDASIVEQKWWCHMQPCLEGEECKVLPDRKGWSCSSGNKVKTTRVTH

SEQ ID NO: 304 - protein, 133 aa, synthetic construct
  REGION 1..133: note = TAFA3_Homo sapiens
MSERVERNWSTGGWLLALCLAWLWTHLTLAALQPPTATVLVQQGTCEVIAAHRCCNRNRIEERSQTVKCSCFSGQVAGTTRAKPSCVDASIVLQRWWCQMEPCLPGEECKVLPDLSGWSCSSGHKVKTTKVTR

SEQ ID NO: 305 - DNA, 405 bp, synthetic construct
  misc_feature 1..405: note = TAFA4_Mus musculus
  source 1..405: mol_type = other DNA
atgagagtctgtgctaagtgggtgctgctgtcacgctggctggttctgacctatgtgttaatggtctgctgtaagctgatgtccgcctcgagccagcacctccggggacatgcaggtcaccacctgatcaagccaggtacctgcgaggtggtcgccgtgcaccgctgctgcaataagaaccgcatagaggagcgctctcagacggtcaaatgttcctgcttcccaggccaggtggctggcacaactcgggcacagccttcttgtgttgaagctgccattgtgattgagaagtggtggtgccacatgaatccttgcttggaaggagaggactgtaaagtgcttccagactcttcgggttggtcctgtagcagtggcaataaagtcaaaaccaccaaggtgacccgg

SEQ ID NO: 306 - DNA, 420 bp, synthetic construct
  misc_feature 1..420: note = TAFA4_Homo sapiens
  source 1..420: mol_type = other DNA
atgaggtccccaaggatgagagtctgtgctaagtcagtgttgctgtcgcactggctctttctagcctacgtgttaatggtgtgctgtaagctgatgtccgcctcaagccagcacctccggggacatgcaggtcaccaccaaatcaagcaagggacctgtgaggtggtcgccgtgcacaggtgctgcaataagaaccgcatagaagagcggtcacaaacggtcaagtgctcttgcttcccgggacaggtggcgggcacaactcgggctcaaccttcttgtgttgaagcttccattgtgattcagaaatggtggtgtcacatgaatccgtgtttggaaggagaggattgtaaagtgctgccagattactcaggttggtcctgtagcagtggcaataaagtcaaaactacgaaggtaacgcgg

SEQ ID NO: 307 - DNA, 405 bp, synthetic construct
  misc_feature 1..405: note = TAFA4_Gekko japonicus
  source 1..405: mol_type = other DNA
atgaggttctgtgccaaatcaatgcttccatctcagtggctgttcctggcatatgtgttaatggtgtgctgtaaatcgttgtccgcgactagctaccatccccgggggcacccaggccaccaccaagttaagcaagggacctgtgaagtggttgcagtgcatctgtgttgcaacaagaacaggattgaagagctgtctcagacaggcaactgttcttgcctcccagggcaagttgcgggtacaacacgaactcagccctcctgtgtggaagccgccattgtcatccagaagtggtggtgtcagatgagcccttgtctggaaggagaggaatgtaaagtgcttcctgattcctcagggtggtcctgcagcagtgggaataaagtcaaaactaccaaggtgacccgg

SEQ ID NO: 308 - DNA, 405 bp, synthetic construct
  misc_feature 1..405: note = TAFA4_Danio rerio
  source 1..405: mol_type = other DNA
atgcagctgtggggtcgatctctgtggccgctgcggattgtgctcttgttcaccttggtaatgtgttcgtgtgggttggtttctgcgggcacgcggagtctgcggggacacacagcttcataccaggtaaagcagggtacctgtgaggtggttgccatccaccgctgctgcaataagaacaagattgaggagcgttcacagaccgtcaagtgctcatgtttccctggtcaggtggccggtaccacacgtgcacagccatcttgtgtggaggcttccatcgtgctacagaagtggtggtgccaaatgcacccatgtttggatggcgaggagtgcaaagctcttccagatctgactggctggtcctgcagcaccggtaacaaagtcaaaaccactaaggtcacacga

SEQ ID NO: 309 - DNA, 399 bp, synthetic construct
  misc_feature 1..399: note = TAFA1_Homo sapiens
  source 1..399: mol_type = other DNA
atggcaatggtctctgcgatgtcctgggtcctgtatttgtggataagtgcttgtgcaatgctactctgccatggatcccttcagcacactttccagcagcatcacctgcacagaccagaaggagggacgtgtgaagtgatagcagcacaccgatgttgtaacaagaatcgcattgaggagcggtcacaaacagtaaagtgttcctgtctacctggaaaagtggctggaacaacaagaaaccggccttcttgcgtcgatgcctccatagtgattgggaaatggtggtgtgagatggagccttgcctagaaggagaagaatgtaagacactccctgacaattctggatggatgtgcgcaacaggcaacaaaattaagaccacgagaattcacccaagaacc

SEQ ID NO: 310 - DNA, 393 bp, synthetic construct
  misc_feature 1..393: note = TAFA2_Homo sapiens
  source 1..393: mol_type = other DNA
atgagtaagagatacttacagaaagcaacaaaaggaaaactgctaataataatatttattgtaaccttgtgggggaaagttgtatccagtgcaaaccatcataaagctcaccatgttaaaacgggaacttgtgaggtggtggcactccacagatgctgtaataagaacaagatagaagaacggtcacaaacagtcaagtgctcctgcttccctgggcaggtggcaggcaccacgcgagctgctccatcatgtgtggatgcttcaatagtggaacagaaatggtggtgccatatgcagccatgtctagagggagaagaatgtaaagttcttccggatcggaaaggatggagctgttcctctgggaataaagtcaaaacaactagggtaacccat

SEQ ID NO: 311 - DNA, 399 bp, synthetic construct
  misc_feature 1..399: note = TAFA3_Homo sapiens
  source 1..399: mol_type = other DNA
atgagtgagagggtcgagcggaactggagcacgggcggctggctgctggcactgtgcctggcctggctgtggacccacctgaccttggctgccttgcagcctcccactgccacagtgcttgtgcagcagggcacctgcgaggtgattgcggctcaccgctgctgcaaccggaaccgcatcgaggagcgctcccagacggtgaaatgctcctgtttttctggccaggtggccggcaccacgcgggcaaagccctcctgcgtggacgcctccatcgtcctgcagagatggtggtgtcagatggagccctgcctgccgggggaggagtgtaaggtgctcccggacctgtcgggatggagctgcagcagtggacacaaagtcaaaaccaccaaggtcacacga

SEQ ID NO: 312 - protein, 19 aa, synthetic construct
  REGION 1..19: note = mIgG heavy chain V region signal peptide
MGWSCIILFLVATATGVHS

SEQ ID NO: 313 - protein, 20 aa, synthetic construct
  REGION 1..20: note = Interleukin2 signal peptide
MYRMQLLSCIALSLALVTNS